European Patent Application EP 4 252 846 A1, published October 4, 2023. Title: Agent for regulating the expression of RPS25 gene and/or the function of RPS25. Applicant: Sumitomo Dainippon Pharma Co., Ltd. Luxna Biotech Co., Ltd. The sequence listing filed with the application follows.

SEQUENCE LISTING (788 sequences)

SEQ ID NO: 1 - DNA, 483 bp, Homo sapiens
ctttttgtccgacatcttgacgaggctgcggtgtctgctgctattctccgagcttcgcaatgccgcctaaggacgacaagaagaagaaggacgctggaaagtcggccaagaaagacaaagacccagtgaacaaatccgggggcaaggccaaaaagaagaagtggtccaaaggcaaagttcgggacaagctcaataacttagtcttgtttgacaaagctacctatgataaactctgtaaggaagttcccaactataaacttataaccccagctgtggtctctgagagactgaagattcgaggctccctggccagggcagcccttcaggagctccttagtaaaggacttatcaaactggtttcaaagcacagagctcaagtaatttacaccagaaataccaagggtggagatgctccagctgctggtgaagatgcatgaataggtccaaccagctgtacatttggaaaaataaaactttattaaa

SEQ ID NO: 2 - DNA, 2637 bp, Homo sapiens
cttcctttttgtccgacatcttgacgaggctgcggtgtctgctgctattctccgagcttcgcaatggtaagcttcaggggtgtgaagtcgccggcgttcttgggtttgaggactcagtggggagagccttcggcgggagcgctccttggcctgccggcctcggttgcagggcgggcgcggttattgcttggcccatgtgctctggtggtggagtttgcgggggctgagggcgcagtattaggggactttggcgctatttgaggacctggttgcattcccgctgccctcctacagccgcctaaggacgacaagaagaagaaggacgctggaaagtcggccaagaaagacaaagacccagtgaacaaatccgggggcaaggccaaaaagaaggtagaaataagacctctctgaaagagactaggggtaactctctcgtaatcctctagtaataggtaacttgtatagtaagtggtttttcaggtgtagatttctagagtcaaaatgtgagagtttatcttcccgtcaccactcgttctttttcccattaggatcatgaaaatgggtctgttgtgcgaagtgtctgccgctgtgcctgctgtgttatttttaactgatctagtggggctcggcccctgtttgaaggccaaaaacgtgtcggtgttttttttttgtttttgttttagtaatgtgtaatttatccttgataacggtggaacagatttctctgacgcagattactcgagagggaaagggtgcttctgccagaaatactaacttgtttctgttttgttttggtgagcagaagtggtccaaaggcaaagttcgggacaagctcaataacttagtcttgtttgacaaagctacctatgataaactctgtaaggaagttcccaactataaacttataaccccagctgtggtctctgagagactgaagattcgaggctccctggccagggcagcccttcaggagctccttagtaaaggtgaggggtgtatcctacatgtgtgtttttgtaggttaaattgtcttgaccatgttaagcatcttcagtggttttgctggaaaagcagaattaaaaaaaaaaagcgtggcttgaccattggctgttagtaatgtaattctgacgtcttactcctgatcctgagatgaattctcagggttcttagccacttttgtgccgtggaccctgtggcagtttagtgaagcccaaggatcttttatgtttcgagtaaatggatgcatagaattacagggacaaccgtttttgaaataattagattactattttgaaacaactttgaaaatgtttaaaacctttatggtaaatattttgttgatgtattaaattttaaaaccagaaatttagtacggtctactcagtagtatggtctgattaccataattccacaataataaggctcagctaactatagtgactgaacgtctataattctagcactttgggaggccaaggcgggtgaatcaacggaggtcaggagttaaagaccagcctggccaatatggtgaaaacctgctctactgaaagttagctggacgtgggggcacacgtctgtaatcccagctactcaggatgctgaggcatgaggatcccttgaacccaggagatggaggtggcagtgagccgagatgacaccactgcactccagccttagtgacagcaaaagactgtctcagaaagggggggggggtggaagataatggagccctaatttaaaggaaaagtaaggatagatgatcgttaaaaactaggattctcggttaccgaacgtcagattaagcaattctggagccaggtgcagtggtacccttgtatttctagctacttgggaggccaaagcaggaggatcatttgagccaaggagttttaagaccattctgggcacctctgagagaactctgtctttttgttttccttttctttaaatagagatgcggttttgccatgttgcccaggctggtctcctgggctcaagagatccacctgtccaaagtgctgggattacaggcatgagcctctgcacccggccaaaacaaaccttactagagtctcattctgttgcccaggttggagtgcggaggggcagtcttggctcaatgcaaccaccaattcctgggttcaggtggtcctcacctcagcttcccaagtagctggaattacaagcatgtgccaccatgcccagctaatttttgtatttttggtagagatggggtttcaccttgttggccaggctggtgtgcaactccttacctcaagctatctgcccgtctccacctcccaaagcagtgggattataagcatgagccaccgcgcccagccaaaaaccttactagtttctattgtagcatctgttaagcatctcatcgtgctattctctccccctaggacttatcaaactggtttcaaagcacagagctcaagtaatttacaccagaaataccaagggtggagatgctccagctgctggtgaagatgcatgaataggtgagtaggaatgtgtgggctcatggtgtaggaggtagatacaaagctttatggttctgattcttttaatttttttttacaggtccaaccagctgtacatttggaaaaataaaactttattaaatcaaat

SEQ ID NO: 3 - DNA, 501 bp, monkey
ctttttgtccgacatcttagcaagccagcggtgtctgctgctgctccccgagcttcgcaatgccgcccaaggacgacaagaagaaggaggacgccggaaagtcggccaagaaagacaaagacccagtgaacaaatctgggggcaaggccaaaaagaagaagtggtccaaaggcaaagttcgggacaagctcaataacttagtcttgtttgacaaagctacctacgacaaactctgtaaggaagttcccaactataaacttataaccccagctgtagtctctgagagactgaagattcgaggctccctggccagggcagcccttcaggagctccttagtaaaggacttatcaaactggtttcaaagcacagagctcaagtaatttacaccagaaataccaagggcggagatgctccagctgctggtgaagatgcatgaataggtccaaccaattgtacatttggaaaaataaaactttattaaatcaaaaaaaaaaaaaaaa

SEQ ID NO: 4 - DNA, 701 bp, mouse
agcgaggctgctgtggtctacacgactctctgagcttcgccatgcctcccaaagacgacaagaagaagaaagatgccggaaagtcggccaaaaaggataaagacccagtaaataaatctggtggcaaggccaagaagaagaagtggtccaaaggcaaagttcgggacaagttgaacaatcttgtcctgttcgacaaagcgacatacgacaagctctgtaaggaggttccgaactataagcttattactccagccgtggtctctgagagactgaagattcgcggttccttggccagggcagcccttcaggagctccttagtaaaggacttatcaagctggtttcaaagcacagagcccaagtaatttacaccagaaacacaaagggtggggacgctccagctgctggcgaagatgcatgaacaggttcaatcagctgtacatttggaaaaataaaactttattgaatcaaatgaatgggtgcatctgtttcctaaggcagccggggaggatttggtcttaggaataatagctggaattggtttgttggccatgaagtcagatgcaattgcgcctgggaaccttcagcttttccctttacgtggttgcttgcttcttgttgcagcttcggttttgaattgatgcctgaaagaaaataaaaacttagcaagactaatggtaaatctaaaaaaaaaaaaaaaaaa

SEQ ID NO: 5 - DNA, 2704 bp, monkey
ctttttgtccgacatcttagcaagccagcggtgtctgctgctgctccccgagcttcgcaatggtaagctacaggggtatgaactcgccggggttcttgggtttgaggactcagtggggagagccttcggcgggagctctccttggcctgccgaccttggttgcagggcgggcgcggttattgcttcgcccatgtgctcggtggtggagtttgcgggggctgagggcgcagtattaggggagtttggggctacttgaggacctggttgcattcccgctgccctcctacagccgcccaaggacgacaagaagaagaaggacgccggaaagtcggccaagaaagacaaagacccagtgaacaaatctgggggcaaggccaaaaagaaggtaggaataagatccctctgagagagactaggggttccctcccgtaaccttctggtaataggtagcttgtatagcaattggtttttcaggtatagatttctagagtaaaaatgtgagagtttatcctcccatcaccattcattctttttcctagtttccattaggatcatgaaaatgagaccagtgtgtaaagtgtctgcctctgtgcctgtcgtgtgatttttaactgatctagtggggctcggcccctgttctgaagcccaagcacctgtcgggttttttttttttttttttagtaatgtgtaatttatctttgatgatgatggaacagatttctctgacgcagattactcgagagggaaagggtgcttctgccagaaatactaacttgtttctgttttgttttggtgagcagaagtggtccaaaggcaaagttcgggacaagctcaataacttagtcttgtttgacaaagctacctacgacaaactctgtaaggaagttcccaactataaacttataaccccagctgtagtctctgagagactgaagattcgaggctccctggccagggcagcccttcaggagctccttagtaaaggtgaggggtgtatcctacatgtgtgcttttgtagggtaaattgtcttgaccacgttaaccatcttcagtgattttgcgggaaaaacagaattaaaaaaaaaaaaaaaaaaaaaaggcatagcttgaccattgactgttagtaatgtaattctgatgtcttactcctgagatgaattcttagggtttgtagccactttcgtgctgtggaccctgtggcagtttggtgaagcccaaggatcttttatgtttcaagtaaatggatgcatagaattacagggacaacaggttttgaaataattagattaatattttaaaacaattttgaaaatgttgaaaacctttatggtaaatattttgatgtattaaattttaaaaccagaaatttagcatggtctactcagtagtatggtttgattaccataattccacaataataagggtcagctaactatagtgactgaacatctgtaattctagcactttggaaggctgaggcgggtgaatcaccggaggtcaggagttcgagaccagcctggccaatatggtgaaaacctgtctttactgaaaatccaaaaattagccggacgtgatggcgcacgcctataatcccagctactcaggatgctgaggcatgaggattgcttgaacccaggagatggaggtggcagtgagccgagatggcactactgcactccagctttggtgacagagcaagagactgtctcaaaaaagggggcggggaggtgcggtggaagataatgggcccctaatttaaaggaaaagtaaagatagatgatcgttaaaaactgtaggattctctgttacgaaacgtcagattaagcaggtgcagtgatacccttgtatttctagctacttgggaggccaaggcaggaggatcatttgagccaaggagtttgagtacattctgggcacctttgagaggacccccctctcccagcctttttttttttcttttaaatagagatgctgttttgctctgttgcccaggctggtctcctgggctcaagagatccacctgtccaaagtgctgggattataggcatgagccactacacctggccaaaacagaaaccttaatagtatgtttttgtttttttttttttggttttttttttttttttttttaaagacagtctcactctgtcgcccaggctggagtgcagaggggcaatcttggctcactgcaaccaccaactcctgggttcaggcagtcctcacacctcagcctcccaagtacctgggattacaaacacgtgccaccatgcctcactaatttttgtatcttcggtagagatggggtttcaccatgttggccaggctggtgtgcaactccttacctcaagctgtctgcccgccttcacctcccaaagtggtgggattacgagcatgagccaccatgcccaaccaaaaaccttactagtttctattatagcatctattaagcatctcatcctactatcttctctccctaggacttatcaaactggtttcaaagcacagagctcaagtaatttacaccagaaataccaagggcggagatgctccagctgctggtgaagatgcatgaataggtgagtaggaatgcgtgggctcatggagtaggaggtagatacaaagctatggttctgattcttgtaattttttttttacaggtccaaccaattgtacatttggaaaaataaaactttattaaatcaaa

SEQ ID NO: 6 - DNA, 2693 bp, mouse
agcgaggctgctgtggtctacacgactctctgagcttcgccatggtaaggcccgcgagggttgagcagtggggttcagaggatcgggcggtgctggggggaggtggaggcgaccctacacggactgcttcgtgacccgcgggcctgcctctccgggcggctgccgccatcgtgtccatgtgctccggcggcggcgcctgggtgggtgaagggctgcgatcggggtgcatgggaccaccatgtgactggcctgcactcccgctttcttcccctagcctcccaaagacgacaagaagaagaaagatgccggaaagtcggccaaaaaggataaagacccagtaaataaatctggtggcaaggccaagaagaaggtaggcgatagctatttgtaatgggaatctgtgggacctgtcgtgaacttgtgctgtaagtttttccccagataccgaattctaaaatcacatagtcactttaagaatacagtggtgtaatacttttataaagtaatggtattaaaccttattaatgttacgacccttttaagatggttccccttttgaccaccagctgtgaaattactatttgttttttcaagatgggtttctctgaatagccctgactgtcctgaactcactctgtagaccaggctggcctcgaacttagaaatctgcctgcctcggcctcccgagtgctgggattaaaggcatgtgccaccactgcccagctcatgaaattatttttttttttatgaaattatttttgttgttgctacttaatagttttgctactgctatgaactgtaaggcatatgtctggtcttcagggtatctgatagcgactccaaagttgccaatgcaataagccaagaagtctctaatttccctgagatgatcgtgacagagctttctcagatgcttgatgttagggagcaaagggatggttctgactggttctcatttgttttgatgagcagaagtggtccaaaggcaaagttcgggacaagttgaacaatcttgtcctgttcgacaaagcgacatacgacaagctctgtaaggaggttccgaactataagcttattactccagccgtggtctctgagagactgaagattcgcggttccttggccagggcagcccttcaggagctccttagtaaaggtaggtgatgtgcccttgttcttaccagtgcattgtcttgttgggagcagtatgactggaaagacttatgaaggatagactgacttccagagtcttaagttttagtaacttcagtgtcctgcattcctttgcagtccttgaattcctggccctttttatttatttatttattgcttctccgttaattgggattaaagtccagagtaccaccttgccttgttattttggaatgccatctcactttgttgtccgggcaaattattctcctgcctctggtgggattttttttgtttgtttgtttttttgtttttcgagacagggtttcctctgtgtagccctggctgtcctggaactcactctgtagaccaggctggccttgaattaagaaatctgcccgcctctgcctcccgagtgctgggattaaaggcgtgcgccaccacgcccggcttggctatagttttaagtacataaacttagcagataggatctaggtgttgttacaagtataaactatggtccttaacatagaggtggtggccccttaagtctgtgccaaggatgtggaagagtttgtgtagttactcctgtaaccacaacacttccatggcaaaatggacttacccaggagctcaggccaactctgcacggcacccgctgtacagcagcgtgagacatactgcctcaacaggatggaagaaaagactgacttcagatagggtgattctctctacgtgcaaatacactaaattattagtaaatcctaaaaacagctacattgatggctggcttgttggtcttcctgtcctagacagagttgggattaagggtacacgcttgtgagcccagcacactgaaggctaaaagggtcagcaccaaatcccaggccggcttggaagttagagtatgacctggcaccctaagaattaaggagttctgtctggaaaagaaataggaaatgtacacttggtatctgctatatgaggaactctggcatccttggagctggagagatgatttccttctcagataccaaatgcacgtgtgtaaggcaagaaccttcaaacactttgaattttctccttaggacttatcaagctggtttcaaagcacagagcccaagtaatttacaccagaaacacaaagggtggggacgctccagctgctggcgaagatgcatgaacaggtgggaagaaaagtttcttggtgtagaagtatcactcgtgccctttatgagatgttgcggttatgactttgtttttttttgtttgttttacaggttcaatcagctgtacatttggaaaaataaaactttattgaatcaaatgaatgggtgcatctgtttcctaaggcagccggggaggatttggtcttaggaataatagctggaattggtttgttggccatgaagtcagatgcaattgcgcctgggaaccttcagcttttccctttacgtggttgcttgcttcttgttgcagcttcggttttgaattgatgcctgaaagaaaataaaaacttagcaagactaatggtaaatcta

SEQ ID NO: 7 - DNA, 15 bp, Artificial Sequence
  h8-22-A ASO for hRPS25 mRNA
  modified_base (1)..(1): m5c
cgtcaagatgtcgga

SEQ ID NO: 8 - DNA, 15 bp, Artificial Sequence
  h9-23-A ASO for hRPS25 mRNA
  modified_base (2)..(2): m5c
  modified_base (13)..(13): m5c
tcgtcaagatgtcgg

SEQ ID NO: 9 - DNA, 15 bp, Artificial Sequence
  h10-24-A ASO for hRPS25 mRNA
  modified_base (1)..(1): m5c
  modified_base (3)..(3): m5c
  modified_base (14)..(14): m5c
ctcgtcaagatgtcg

SEQ ID NO: 10 - DNA, 15 bp, Artificial Sequence
  h27-41-A ASO for hRPS25 mRNA
  modified_base (2)..(2): m5c
  modified_base (14)..(14): m5c
gcagcagacaccgca

SEQ ID NO: 11 - DNA, 15 bp, Artificial Sequence
  h28-42-A ASO for hRPS25 mRNA
  modified_base (3)..(3): m5c
  modified_base (13)..(13): m5c
agcagcagacaccgc

SEQ ID NO: 12 - DNA, 15 bp, Artificial Sequence
  h29-43-A ASO for hRPS25 mRNA
  modified_base (13)..(13): m5c
  modified_base (14)..(14): m5c
tagcagcagacaccg

SEQ ID NO: 13 - DNA, 15 bp, Artificial Sequence
  h30-44-A ASO for hRPS25 mRNA
  modified_base (14)..(14): m5c
atagcagcagacacc

SEQ ID NO: 14 - DNA, 15 bp, Artificial Sequence
  h32-46-A ASO for hRPS25 mRNA
  modified_base (14)..(14): m5c
gaatagcagcagaca

SEQ ID NO: 15 - DNA, 15 bp, Artificial Sequence
  h33-47-A ASO for hRPS25 mRNA
agaatagcagcagac

SEQ ID NO: 16 - DNA, 15 bp, Artificial Sequence
  h34-48-A ASO for hRPS25 mRNA
gagaatagcagcaga

SEQ ID NO: 17 - DNA, 15 bp, Artificial Sequence
  h35-49-A ASO for hRPS25 mRNA
  modified_base (13)..(13): m5c
ggagaatagcagcag

SEQ ID NO: 18 - DNA, 15 bp, Artificial Sequence
  h36-50-A ASO for hRPS25 mRNA
  modified_base (1)..(1): m5c
  modified_base (14)..(14): m5c
cggagaatagcagca

SEQ ID NO: 19 - DNA, 15 bp, Artificial Sequence
  h37-51-A ASO for hRPS25 mRNA
  modified_base (2)..(2): m5c
tcggagaatagcagc

SEQ ID NO: 20 - DNA, 15 bp, Artificial Sequence
  h38-52-A ASO for hRPS25 mRNA
  modified_base (1)..(1): m5c
  modified_base (3)..(3): m5c
  modified_base (13)..(13): m5c
ctcggagaatagcag

SEQ ID NO: 21 - DNA, 15 bp, Artificial Sequence
  h72-86-A ASO for hRPS25 mRNA
  modified_base (1)..(1): m5c
cttcttcttgtcgtc

SEQ ID NO: 22 - DNA, 15 bp, Artificial Sequence
  h79-93-A ASO for hRPS25 mRNA
  modified_base (1)..(1): m5c
  modified_base (14)..(14): m5c
cgtccttcttcttct

SEQ ID NO: 23 - DNA, 15 bp, Artificial Sequence
  h101-115-A ASO for hRPS25 mRNA
  modified_base (2)..(2): m5c
tctttcttggccgac

SEQ ID NO: 24 - DNA, 15 bp, Artificial Sequence
  h102-116-A ASO for hRPS25 mRNA
  modified_base (3)..(3): m5c
  modified_base (13)..(13): m5c
gtctttcttggccga

SEQ ID NO: 25 - DNA, 15 bp, Artificial Sequence
  h103-117-A ASO for hRPS25 mRNA
  modified_base (13)..(13): m5c
  modified_base (14)..(14): m5c
tgtctttcttggccg

SEQ ID NO: 26 - DNA, 15 bp, Artificial Sequence
  h122-136-A ASO for hRPS25 mRNA
gatttgttcactggg

SEQ ID NO: 27 - DNA, 15 bp, Artificial Sequence
  h124-138-A ASO for hRPS25 mRNA
  modified_base (1)..(1): m5c
  modified_base (13)..(13): m5c
cggatttgttcactg

SEQ ID NO: 28 - DNA, 15 bp, Artificial Sequence
  h125-139-A ASO for hRPS25 mRNA
  modified_base (1)..(1): m5c
  modified_base (2)..(2): m5c
  modified_base (14)..(14): m5c
ccggatttgttcact

SEQ ID NO: 29 - DNA, 15 bp, Artificial Sequence
  h126-140-A ASO for hRPS25 mRNA
  modified_base (1)..(1): m5c
  modified_base (2)..(2): m5c
  modified_base (3)..(3): m5c
  modified_base (13)..(13): m5c
cccggatttgttcac

SEQ ID NO: 30 - DNA, 15 bp, Artificial Sequence
  h140-154-A ASO for hRPS25 mRNA
  modified_base (13)..(13): m5c
  modified_base (14)..(14): m5c
tttttggccttgccc

SEQ ID NO: 31 - DNA, 15 bp, Artificial Sequence
  h160-174-A ASO for hRPS25 mRNA
  modified_base (3)..(3): m5c
  modified_base (14)..(14): m5c
tgcctttggaccact

SEQ ID NO: 32 - DNA, 15 bp, Artificial Sequence
  h161-175-A ASO for hRPS25 mRNA
  modified_base (13)..(13): m5c
ttgcctttggaccac

SEQ ID NO: 33 - DNA, 15 bp, Artificial Sequence
  h180-194-A ASO for hRPS25 mRNA
  modified_base (13)..(13): m5c
  modified_base (14)..(14): m5c
attgagcttgtcccg

SEQ ID NO: 34 - DNA, 15 bp, Artificial Sequence
  h181-195-A ASO for hRPS25 mRNA
  modified_base (13)..(13): m5c
  modified_base (14)..(14): m5c
tattgagcttgtccc

SEQ ID NO: 35 - DNA, 15 bp, Artificial Sequence
  h182-196-A ASO for hRPS25 mRNA
  modified_base (14)..(14): m5c
ttattgagcttgtcc

SEQ ID NO: 36 - DNA, 15 bp, Artificial Sequence
  h183-197-A ASO for hRPS25 mRNA
gttattgagcttgtc

SEQ ID NO: 37 - DNA, 15 bp, Artificial Sequence
  h184-198-A ASO for hRPS25 mRNA
agttattgagcttgt

SEQ ID NO: 38 - DNA, 15 bp, Artificial Sequence
  h187-201-A ASO for hRPS25 mRNA
  modified_base (1)..(1): m5c
  modified_base (14)..(14): m5c
ctaagttattgagct

SEQ ID NO: 39 - DNA, 15 bp, Artificial Sequence
  h188-202-A ASO for hRPS25 mRNA
  modified_base (2)..(2): m5c
actaagttattgagc

SEQ ID NO: 40 - DNA, 15 bp, Artificial Sequence
  h189-203-A ASO for hRPS25 mRNA
  modified_base (3)..(3): m5c
gactaagttattgag

SEQ ID NO: 41 - DNA, 15 bp, Artificial Sequence
  h191-205-A ASO for hRPS25 mRNA
aagactaagttattg

SEQ ID NO: 42 - DNA, 15 bp, Artificial Sequence
  h193-207-A ASO for hRPS25 mRNA
  modified_base (2)..(2): m5c
acaagactaagttat

SEQ ID NO: 43 - DNA, 15 bp, Artificial Sequence
  h196-210-A ASO for hRPS25 mRNA
  modified_base (1)..(1): m5c
caaacaagactaagt

SEQ ID NO: 44 - DNA, 15 bp, Artificial Sequence
  h197-211-A ASO for hRPS25 mRNA
  modified_base (2)..(2): m5c
tcaaacaagactaag

SEQ ID NO: 45 - DNA, 15 bp, Artificial Sequence
  h208-222-A ASO for hRPS25 mRNA
  modified_base (13)..(13): m5c
aggtagctttgtcaa

SEQ ID NO: 46 - DNA, 15 bp, Artificial Sequence
  h209-223-A ASO for hRPS25 mRNA
  modified_base (14)..(14): m5c
taggtagctttgtca

SEQ ID NO: 47 - DNA, 15 bp, Artificial Sequence
  h210-224-A ASO for hRPS25 mRNA
ataggtagctttgtc

SEQ ID NO: 48 - DNA, 15 bp, Artificial Sequence
  h213-227-A ASO for hRPS25 mRNA
  modified_base (3)..(3): m5c
atcataggtagcttt

SEQ ID NO: 49 - DNA, 15 bp, Artificial Sequence
  h214-228-A ASO for hRPS25 mRNA
  modified_base (13)..(13): m5c
tatcataggtagctt

SEQ ID NO: 50 - DNA, 15 bp, Artificial Sequence
  h216-230-A ASO for hRPS25 mRNA
tttatcataggtagc

SEQ ID NO: 51 - DNA, 15 bp, Artificial Sequence
  h217-231-A ASO for hRPS25 mRNA
gtttatcataggtag

SEQ ID NO: 52 - DNA, 15 bp, Artificial Sequence
  h219-233-A ASO for hRPS25 mRNA
gagtttatcataggt

SEQ ID NO: 53 - DNA, 15 bp, Artificial Sequence
  h220-234-A ASO for hRPS25 mRNA
agagtttatcatagg

SEQ ID NO: 54 - DNA, 15 bp, Artificial Sequence
  h242-256-A ASO for hRPS25 mRNA
  modified_base (14)..(14): m5c
ttatagttgggaact

SEQ ID NO: 55 - DNA, 15 bp, Artificial Sequence
  h243-257-A ASO for hRPS25 mRNA
tttatagttgggaac

SEQ ID NO: 56 - DNA, 15 bp, Artificial Sequence
  h253-267-A ASO for hRPS25 mRNA
gggttataagtttat

SEQ ID NO: 57 - DNA, 15 bp, Artificial Sequence
  h254-268-A ASO for hRPS25 mRNA
ggggttataagttta

SEQ ID NO: 58 - DNA, 15 bp, Artificial Sequence
  h259-273-A ASO for hRPS25 mRNA
  modified_base (1)..(1): m5c
cagctggggttataa

SEQ ID NO: 59 - DNA, 15 bp, Artificial Sequence
  h260-274-A ASO for hRPS25 mRNA
  modified_base (2)..(2): m5c
acagctggggttata

SEQ ID NO: 60 - DNA, 15 bp, Artificial Sequence
  h261-275-A ASO for hRPS25 mRNA
  modified_base (1)..(1): m5c
  modified_base (3)..(3): m5c
cacagctggggttat

SEQ ID NO: 61 - DNA, 15 bp, Artificial Sequence
  h285-299-A ASO for hRPS25 mRNA
  modified_base (2)..(2): m5c
  modified_base (14)..(14): m5c
tcgaatcttcagtct

SEQ ID NO: 62 - DNA, 15 bp, Artificial Sequence
  h286-300-A ASO for hRPS25 mRNA
  modified_base (1)..(1): m5c
  modified_base (3)..(3): m5c
ctcgaatcttcagtc

SEQ ID NO: 63 - DNA, 15 bp, Artificial Sequence
  h295-309-A ASO for hRPS25 mRNA
  modified_base (1)..(1): m5c
  modified_base (2)..(2): m5c
ccagggagcctcgaa

SEQ ID NO: 64 - DNA, 15 bp, Artificial Sequence
  h296-310-A ASO for hRPS25 mRNA
  modified_base (2)..(2): m5c
  modified_base (3)..(3): m5c
  modified_base (13)..(13): m5c
gccagggagcctcga

SEQ ID NO: 65 - DNA, 15 bp, Artificial Sequence
  h297-311-A ASO for hRPS25 mRNA
  modified_base (3)..(3): m5c
  modified_base (14)..(14): m5c
ggccagggagcctcg

SEQ ID NO: 66 - DNA, 15 bp, Artificial Sequence
  h325-339-A ASO for hRPS25 mRNA
  modified_base (3)..(3): m5c
  modified_base (13)..(13): m5c
  modified_base (14)..(14): m5c
tactaaggagctcct

SEQ ID NO: 67 - DNA, 15 bp, Artificial Sequence
  h326-340-A ASO for hRPS25 mRNA
  modified_base (14)..(14): m5c
ttactaaggagctcc

SEQ ID NO: 68 - DNA, 15 bp, Artificial Sequence
  h327-341-A ASO for hRPS25 mRNA
  modified_base (13)..(13): m5c
tttactaaggagctc

SEQ ID NO: 69 - DNA, 15 bp, Artificial Sequence
  h340-354-A ASO for hRPS25 mRNA
  modified_base (13)..(13): m5c
gtttgataagtcctt

SEQ ID NO: 70 - DNA, 15 bp, Artificial Sequence
  h341-355-A ASO for hRPS25 mRNA
  modified_base (13)..(13): m5c
  modified_base (14)..(14): m5c
agtttgataagtcct

SEQ ID NO: 71 - DNA, 15 bp, Artificial Sequence
  h342-356-A ASO for hRPS25 mRNA
  modified_base (1)..(1): m5c
  modified_base (14)..(14): m5c
cagtttgataagtcc

SEQ ID NO: 72 - DNA, 15 bp, Artificial Sequence
  h343-357-A ASO for hRPS25 mRNA
  modified_base (1)..(1): m5c
  modified_base (2)..(2): m5c
ccagtttgataagtc

SEQ ID NO: 73 - DNA, 15 bp, Artificial Sequence
  h344-358-A ASO for hRPS25 mRNA
  modified_base (2)..(2): m5c
  modified_base (3)..(3): m5c
accagtttgataagt

SEQ ID NO: 74 - DNA, 15 bp, Artificial Sequence
  h365-379-A ASO for hRPS25 mRNA
  modified_base (2)..(2): m5c
acttgagctctgtgc

SEQ ID NO: 75 - DNA, 15 bp, Artificial Sequence
  h375-389-A ASO for hRPS25 mRNA
ggtgtaaattacttg

SEQ ID NO: 76 - DNA, 15 bp, Artificial Sequence
  h390-404-A ASO for hRPS25 mRNA
  modified_base (2)..(2): m5c
  modified_base (3)..(3): m5c
  modified_base (14)..(14): m5c
acccttggtatttct

SEQ ID NO: 77 - DNA, 15 bp, Artificial Sequence
  h393-407-A ASO for hRPS25 mRNA
  modified_base (2)..(2): m5c
  modified_base (3)..(3): m5c
tccacccttggtatt

SEQ ID NO: 78 - DNA, 15 bp, Artificial Sequence
  h394-408-A ASO for hRPS25 mRNA
  modified_base (1)..(1): m5c
  modified_base (3)..(3): m5c
ctccacccttggtat

SEQ ID NO: 79 - DNA, 15 bp, Artificial Sequence
  h430-444-A ASO for hRPS25 mRNA
  modified_base (3)..(3): m5c
  modified_base (13)..(13): m5c
gacctattcatgcat

SEQ ID NO: 80 - DNA, 15 bp, Artificial Sequence
  h431-445-A ASO for hRPS25 mRNA
  modified_base (14)..(14): m5c
ggacctattcatgca

SEQ ID NO: 81 - DNA, 15 bp, Artificial Sequence
  h432-446-A ASO for hRPS25 mRNA
tggacctattcatgc

SEQ ID NO: 82 - DNA, 15 bp, Artificial Sequence
  h433-447-A ASO for hRPS25 mRNA
ttggacctattcatg

SEQ ID NO: 83 - DNA, 15 bp, Artificial Sequence
  h434-448-A ASO for hRPS25 mRNA
  modified_base (13)..(13): m5c
gttggacctattcat

SEQ ID NO: 84 - DNA, 15 bp, Artificial Sequence
  h435-449-A ASO for hRPS25 mRNA
  modified_base (14)..(14): m5c
ggttggacctattca

SEQ ID NO: 85 - DNA, 15 bp, Artificial Sequence
  h436-450-A ASO for hRPS25 mRNA
tggttggacctattc

SEQ ID NO: 86 - DNA, 15 bp, Artificial Sequence
  h438-452-A ASO for hRPS25 mRNA
  modified_base (2)..(2): m5c
gctggttggacctat

SEQ ID NO: 87 - DNA, 15 bp, Artificial Sequence
  h439-453-A ASO for hRPS25 mRNA
  modified_base (3)..(3): m5c
  modified_base (13)..(13): m5c
agctggttggaccta

SEQ ID NO: 88 - DNA, 15 bp, Artificial Sequence
  h440-454-A ASO for hRPS25 mRNA
  modified_base (1)..(1): m5c
  modified_base (13)..(13): m5c
  modified_base (14)..(14): m5c
cagctggttggacct

SEQ ID NO: 89 - DNA, 15 bp, Artificial Sequence
  h441-455-A ASO for hRPS25 mRNA
  modified_base (2)..(2): m5c
  modified_base (14)..(14): m5c
acagctggttggacc

SEQ ID NO: 90 - DNA, 15 bp, Artificial Sequence
  h442-456-A ASO for hRPS25 mRNA
  modified_base (3)..(3): m5c
tacagctggttggac

SEQ ID NO: 91 - DNA, 15 bp, Artificial Sequence
  h444-458-A ASO for hRPS25 mRNA
tgtacagctggttgg

SEQ ID NO: 92 - DNA, 15 bp, Artificial Sequence
  h446-460-A ASO for hRPS25 mRNA
aatgtacagctggtt

SEQ ID NO: 93 - DNA, 15 bp, Artificial Sequence
  h447-461-A ASO for hRPS25 mRNA
aaatgtacagctggt

SEQ ID NO: 94 - DNA, 15 bp, Artificial Sequence
  h451-465-A ASO for hRPS25 mRNA
  modified_base (3)..(3): m5c
ttccaaatgtacagc

SEQ ID NO: 95 - DNA, 15 bp, Artificial Sequence
  h125-139-B ASO for hRPS25 mRNA
  modified_base (1)..(1): m5c
  modified_base (2)..(2): m5c
  modified_base (14)..(14): m5c
ccggatttgttcact

SEQ ID NO: 96 - DNA, 15 bp, Artificial Sequence
  h125-139-C ASO for hRPS25 mRNA
  modified_base (1)..(1): m5c
  modified_base (2)..(2): m5c
  modified_base (14)..(14): m5c
ccggatttgttcact

SEQ ID NO: 97 - DNA, 17 bp, Artificial Sequence
  h124-140-A ASO for hRPS25 mRNA
  modified_base (1)..(1): m5c
  modified_base (2)..(2): m5c
  modified_base (3)..(3): m5c
  modified_base (15)..(15): m5c
cccggatttgttcactg

SEQ ID NO: 98 - DNA, 17 bp, Artificial Sequence
  h124-140-B ASO for hRPS25 mRNA
  modified_base (1)..(1): m5c
  modified_base (2)..(2): m5c
  modified_base (3)..(3): m5c
  modified_base (15)..(15): m5c
cccggatttgttcactg

SEQ ID NO: 99 - DNA, 19 bp, Artificial Sequence
  h123-141-A ASO for hRPS25 mRNA
  modified_base (1)..(1): m5c
  modified_base (2)..(2): m5c
  modified_base (3)..(3): m5c
ccccggatttgttcactgg

SEQ ID NO: 100 - DNA, 19 bp, Artificial Sequence
  h123-141-B ASO for hRPS25 mRNA
  modified_base (1)..(1): m5c
  modified_base (2)..(2): m5c
  modified_base (3)..(3): m5c
ccccggatttgttcactgg

SEQ ID NO: 101 - DNA, 15 bp, Artificial Sequence
  h187-201-B ASO for hRPS25 mRNA
  modified_base (1)..(1): m5c
  modified_base (14)..(14): m5c
ctaagttattgagct

SEQ ID NO: 102 - DNA, 15 bp, Artificial Sequence
  h187-201-C ASO for hRPS25 mRNA
  modified_base (1)..(1): m5c
  modified_base (14)..(14): m5c
ctaagttattgagct

SEQ ID NO: 103 - DNA, 17 bp, Artificial Sequence
  h186-202-A ASO for hRPS25 mRNA
  modified_base (2)..(2): m5c
  modified_base (15)..(15): m5c
actaagttattgagctt

SEQ ID NO: 104 - DNA, 17 bp, Artificial Sequence
  h186-202-B ASO for hRPS25 mRNA
  modified_base (2)..(2): m5c
  modified_base (15)..(15): m5c
actaagttattgagctt

SEQ ID NO: 105 - DNA, 19 bp, Artificial Sequence
  h185-203-A ASO for hRPS25 mRNA
  modified_base (3)..(3): m5c
gactaagttattgagcttg

SEQ ID NO: 106 - DNA, 19 bp, Artificial Sequence
  h185-203-B ASO for hRPS25 mRNA
  modified_base (3)..(3): m5c
gactaagttattgagcttg

SEQ ID NO: 107 - DNA, 15 bp, Artificial Sequence
  h213-227-B ASO for hRPS25 mRNA
  modified_base (3)..(3): m5c
atcataggtagcttt

SEQ ID NO: 108 - DNA, 15 bp, Artificial Sequence
  h213-227-C ASO for hRPS25 mRNA
  modified_base (3)..(3): m5c
atcataggtagcttt

SEQ ID NO: 109 - DNA, 17 bp, Artificial Sequence
  h212-228-A ASO for hRPS25 mRNA
tatcataggtagctttg

SEQ ID NO: 110 - DNA, 17 bp, Artificial Sequence
  h212-228-B ASO for hRPS25 mRNA
tatcataggtagctttg

SEQ ID NO: 111 - DNA, 19 bp, Artificial Sequence
  h211-229-A ASO for hRPS25 mRNA
ttatcataggtagctttgt

SEQ ID NO: 112 - DNA, 19 bp, Artificial Sequence
  h211-229-B ASO for hRPS25 mRNA
ttatcataggtagctttgt

SEQ ID NO: 113 - DNA, 15 bp, Artificial Sequence
  h326-340-B ASO for hRPS25 mRNA
  modified_base (14)..(14): m5c
  modified_base (15)..(15): m5c
ttactaaggagctcc

SEQ ID NO: 114 - DNA, 15 bp, Artificial Sequence
  h326-340-C ASO for hRPS25 mRNA
  modified_base (14)..(14): m5c
  modified_base (15)..(15): m5c
ttactaaggagctcc

SEQ ID NO: 115 - DNA, 17 bp, Artificial Sequence
  h325-341-A ASO for hRPS25 mRNA
  modified_base (15)..(15): m5c
  modified_base (16)..(16): m5c
tttactaaggagctcct

SEQ ID NO: 116 - DNA, 17 bp, Artificial Sequence
  h325-341-B ASO for hRPS25 mRNA
  modified_base (15)..(15): m5c
  modified_base (16)..(16): m5c
tttactaaggagctcct

SEQ ID NO: 117 - DNA, 19 bp, Artificial Sequence
  h324-342-A ASO for hRPS25 mRNA
  modified_base (1)..(1): m5c
  modified_base (17)..(17): m5c
ctttactaaggagctcctg

SEQ ID NO: 118 - DNA, 19 bp, Artificial Sequence
  h324-342-B ASO for hRPS25 mRNA
  modified_base (1)..(1): m5c
  modified_base (17)..(17): m5c
ctttactaaggagctcctg

SEQ ID NO: 119 - DNA, 15 bp, Artificial Sequence
  h444-458-B ASO for hRPS25 mRNA
tgtacagctggttgg

SEQ ID NO: 120 - DNA, 15 bp, Artificial Sequence
  h444-458-C ASO for hRPS25 mRNA
tgtacagctggttgg

SEQ ID NO: 121 - DNA, 17 bp, Artificial Sequence
  h442-458-A ASO for hRPS25 mRNA
  modified_base (17)..(17): m5c
tgtacagctggttggac

SEQ ID NO: 122 - DNA, 17 bp, Artificial Sequence
  h442-458-B ASO for hRPS25 mRNA
  modified_base (17)..(17): m5c
tgtacagctggttggac

SEQ ID NO: 123 - DNA, 19 bp, Artificial Sequence
  h442-460-A ASO for hRPS25 mRNA
  modified_base (19)..(19): m5c
aatgtacagctggttggac

SEQ ID NO: 124 - DNA, 19 bp, Artificial Sequence
  h442-460-B ASO for hRPS25 mRNA
  modified_base (19)..(19): m5c
aatgtacagctggttggac

SEQ ID NO: 125 - DNA, 15 bp, Artificial Sequence
  h451-465-B ASO for hRPS25 mRNA
  modified_base (3)..(3): m5c
  modified_base (15)..(15): m5c
ttccaaatgtacagc

SEQ ID NO: 126 - DNA, 15 bp, Artificial Sequence
  h451-465-C ASO for hRPS25 mRNA
  modified_base (3)..(3): m5c
  modified_base (15)..(15): m5c
ttccaaatgtacagc

SEQ ID NO: 127 - DNA, 17 bp, Artificial Sequence
  h450-466-A ASO for hRPS25 mRNA
  modified_base (16)..(16): m5c
tttccaaatgtacagct

SEQ ID NO: 128 - DNA, 17 bp, Artificial Sequence
  h450-466-B ASO for hRPS25 mRNA
  modified_base (16)..(16): m5c
tttccaaatgtacagct

SEQ ID NO: 129 - DNA, 19 bp, Artificial Sequence
  h449-467-A ASO for hRPS25 mRNA
  modified_base (17)..(17): m5c
ttttccaaatgtacagctg

SEQ ID NO: 130 - DNA, 19 bp, Artificial Sequence
  h449-467-B ASO for hRPS25 mRNA
  modified_base (17)..(17): m5c
ttttccaaatgtacagctg

SEQ ID NO: 131 - DNA, 15 bp, Artificial Sequence
  h39-53-A ASO for hRPS25 mRNA
  modified_base (2)..(2): m5c
  modified_base (14)..(14): m5c
gctcggagaatagca

SEQ ID NO: 132 - DNA, 15 bp, Artificial Sequence
  h40-54-A ASO for hRPS25 mRNA
  modified_base (3)..(3): m5c
agctcggagaatagc

SEQ ID NO: 133 - DNA, 15 bp, Artificial Sequence
  h98-112-A ASO for hRPS25 mRNA
  modified_base (3)..(3): m5c
ttcttggccgacttt

SEQ ID NO: 134 - DNA, 15 bp, Artificial Sequence
  h99-113-A ASO for hRPS25 mRNA
  modified_base (13)..(13): m5c
tttcttggccgactt

SEQ ID NO: 135 - DNA, 15 bp, Artificial Sequence
  h100-114-A ASO for hRPS25 mRNA
  modified_base (1)..(1): m5c
  modified_base (14)..(14): m5c
ctttcttggccgact

SEQ ID NO: 136 - DNA, 15 bp, Artificial Sequence
  h104-118-A ASO for hRPS25 mRNA
  modified_base (14)..(14): m5c
ttgtctttcttggcc

SEQ ID NO: 137 - DNA, 15 bp, Artificial Sequence
  h105-119-A ASO for hRPS25 mRNA
tttgtctttcttggc

SEQ ID NO: 138 - DNA, 15 bp, Artificial Sequence
  h106-120-A ASO for hRPS25 mRNA
  modified_base (1)..(1): m5c
ctttgtctttcttgg

SEQ ID NO: 139 - DNA, 15 bp, Artificial Sequence
  h107-121-A ASO for hRPS25 mRNA
  modified_base (2)..(2): m5c
tctttgtctttcttg

SEQ ID NO: 140 - DNA, 15 bp, Artificial Sequence
  h123-137-C ASO for hRPS25 mRNA
ggatttgttcactgg

SEQ ID NO: 141 - DNA, 15 bp, Artificial Sequence
  h127-141-A ASO for hRPS25 mRNA
  modified_base (1)..(1): m5c
  modified_base (2)..(2): m5c
  modified_base (3)..(3): m5c
  modified_base (14)..(14): m5c
ccccggatttgttca

SEQ ID NO: 142 - DNA, 15 bp, Artificial Sequence
  h128-142-A ASO for hRPS25 mRNA
  modified_base (1)..(1): m5c
  modified_base (2)..(2): m5c
  modified_base (3)..(3): m5c
cccccggatttgttc

SEQ ID NO: 143 - DNA, 15 bp, Artificial Sequence
  h129-143-A ASO for hRPS25 mRNA
  modified_base (2)..(2): m5c
  modified_base (3)..(3): m5c
gcccccggatttgtt

SEQ ID NO: 144 - DNA, 15 bp, Artificial Sequence
  h130-144-A ASO for hRPS25 mRNA
  modified_base (3)..(3): m5c
tgcccccggatttgt

SEQ ID NO: 145 - DNA, 15 bp, Artificial Sequence
  h185-199-C ASO for hRPS25 mRNA
aagttattgagcttg

SEQ ID NO: 146 - DNA, 15 bp, Artificial Sequence
  h186-200-C ASO for hRPS25 mRNA
  modified_base (13)..(13): m5c
taagttattgagctt

SEQ ID NO: 147 - DNA, 15 bp, Artificial Sequence
  h190-204-A ASO for hRPS25 mRNA
agactaagttattga

SEQ ID NO: 148 - DNA, 15 bp, Artificial Sequence
  h211-225-A ASO for hRPS25 mRNA
  modified_base (1)..(1): m5c
cataggtagctttgt

SEQ ID NO: 149 - DNA, 15 bp, Artificial Sequence
  h212-226-A ASO for hRPS25 mRNA
  modified_base (2)..(2): m5c
tcataggtagctttg

SEQ ID NO: 150 - DNA, 15 bp, Artificial Sequence
  h215-229-A ASO for hRPS25 mRNA
  modified_base (14)..(14): m5c
ttatcataggtagct

SEQ ID NO: 151 - DNA, 15 bp, Artificial Sequence
  h218-232-A ASO for hRPS25 mRNA
agtttatcataggta

SEQ ID NO: 152 - DNA, 15 bp, Artificial Sequence
  h221-235-A ASO for hRPS25 mRNA
  modified_base (1)..(1): m5c
cagagtttatcatag

SEQ ID NO: 153 - DNA, 15 bp, Artificial Sequence
  h222-236-A ASO for hRPS25 mRNA
  modified_base (2)..(2): m5c
acagagtttatcata

SEQ ID NO: 154 - DNA, 15 bp, Artificial Sequence
  h223-237-A ASO for hRPS25 mRNA
  modified_base (3)..(3): m5c
  modified_base (13)..(13): m5c
tacagagtttatcat

SEQ ID NO: 155 - DNA, 15 bp, Artificial Sequence
  h224-238-A ASO for hRPS25 mRNA
  modified_base (14)..(14): m5c
ttacagagtttatca

SEQ ID NO: 156 - DNA, 15 bp, Artificial Sequence
  h255-269-A ASO for hRPS25 mRNA
tggggttataagttt

SEQ ID NO: 157 - DNA, 15 bp, Artificial Sequence
  h256-270-A ASO for hRPS25 mRNA
  modified_base (1)..(1): m5c
ctggggttataagtt

SEQ ID NO: 158 - DNA, 15 bp, Artificial Sequence
  h257-271-A ASO for hRPS25 mRNA
  modified_base (2)..(2): m5c
gctggggttataagt

SEQ ID NO: 159 - DNA, 15 bp, Artificial Sequence
  h258-272-A ASO for hRPS25 mRNA
  modified_base (3)..(3): m5c
agctggggttataag

SEQ ID NO: 160 - DNA, 15 bp, Artificial Sequence
  h262-276-A ASO for hRPS25 mRNA
  modified_base (1)..(1): m5c
  modified_base (2)..(2): m5c
ccacagctggggtta

SEQ ID NO: 161 - DNA, 15 bp, Artificial Sequence
  h263-277-A ASO for hRPS25 mRNA
  modified_base (2)..(2): m5c
  modified_base (3)..(3): m5c
accacagctggggtt

SEQ ID NO: 162 - DNA, 15 bp, Artificial Sequence
  h264-278-A ASO for hRPS25 mRNA
  modified_base (3)..(3): m5c
gaccacagctggggt

SEQ ID NO: 163 - DNA, 15 bp, Artificial Sequence
  h291-305-A ASO for hRPS25 mRNA
  modified_base (13)..(13): m5c
ggagcctcgaatctt

SEQ ID NO: 164 - DNA, 15 bp, Artificial Sequence
  h292-306-A ASO for hRPS25 mRNA
  modified_base (14)..(14): m5c
gggagcctcgaatct

SEQ ID NO: 165 - DNA, 15 bp, Artificial Sequence
  h293-307-A ASO for hRPS25 mRNA
agggagcctcgaatc

SEQ ID NO: 166 - DNA, 15 bp, Artificial Sequence
  h294-308-A ASO for hRPS25 mRNA
  modified_base (1)..(1): m5c
cagggagcctcgaat

SEQ ID NO: 167 - DNA, 15 bp, Artificial Sequence
  h298-312-A ASO for hRPS25 mRNA
  modified_base (13)..(13): m5c
tggccagggagcctc

SEQ ID NO: 168 - DNA, 15 bp, Artificial Sequence
  h299-313-A ASO for hRPS25 mRNA
  modified_base (1)..(1): m5c
  modified_base (13)..(13): m5c
  modified_base (14)..(14): m5c
ctggccagggagcct

SEQ ID NO: 169 - DNA, 15 bp, Artificial Sequence
  h300-314-A ASO for hRPS25 mRNA
  modified_base (1)..(1): m5c
  modified_base (2)..(2): m5c
  modified_base (14)..(14): m5c
cctggccagggagcc

SEQ ID NO: 170 - DNA, 15 bp, Artificial Sequence
  h321-335-A ASO for hRPS25 mRNA
aaggagctcctgaag

SEQ ID NO: 171 - DNA, 15 bp, Artificial Sequence
  h322-336-A ASO for hRPS25 mRNA
taaggagctcctgaa

SEQ ID NO: 172 - DNA, 15 bp, Artificial Sequence
  h323-337-A ASO for hRPS25 mRNA
  modified_base (1)..(1): m5c
ctaaggagctcctga

SEQ ID NO: 173 - DNA, 15 bp, Artificial Sequence
  h324-338-A ASO for hRPS25 mRNA
  modified_base (2)..(2): m5c
  modified_base (13)..(13): m5c
actaaggagctcctg

SEQ ID NO: 174 - DNA, 15 bp, Artificial Sequence
  h328-342-A ASO for hRPS25 mRNA
  modified_base (1)..(1): m5c
  modified_base (14)..(14): m5c
ctttactaaggagct

SEQ ID NO: 175 - DNA, 15 bp, Artificial Sequence
  h329-343-A ASO for hRPS25 mRNA
  modified_base (1)..(1): m5c
  modified_base (2)..(2): m5c
cctttactaaggagc

SEQ ID NO: 176 - DNA, 15 bp, Artificial Sequence
  h330-344-A ASO for hRPS25 mRNA
  modified_base (2)..(2): m5c
  modified_base (3)..(3): m5c
tcctttactaaggag

SEQ ID NO: 177 - DNA, 15 bp, Artificial Sequence
  h331-345-A ASO for hRPS25 mRNA
  modified_base (3)..(3): m5c
gtcctttactaagga

SEQ ID NO: 178 - DNA, 15 bp, Artificial Sequence
  h426-440-A ASO for hRPS25 mRNA
tattcatgcatcttc

SEQ ID NO: 179 - DNA, 15 bp, Artificial Sequence
  h427-441-A ASO for hRPS25 mRNA
  modified_base (1)..(1): m5c
  modified_base (13)..(13): m5c
ctattcatgcatctt

SEQ ID NO: 180 - DNA, 15 bp, Artificial Sequence
  h428-442-A ASO for hRPS25 mRNA
  modified_base (1)..(1): m5c
  modified_base (2)..(2): m5c
  modified_base (14)..(14): m5c
cctattcatgcatct

SEQ ID NO: 181 - DNA, 15 bp, Artificial Sequence
  h429-443-A ASO for hRPS25 mRNA
  modified_base (2)..(2): m5c
  modified_base (3)..(3): m5c
acctattcatgcatc

SEQ ID NO: 182 - DNA, 15 bp, Artificial Sequence
  h437-451-A ASO for hRPS25 mRNA
  modified_base (1)..(1): m5c
ctggttggacctatt

SEQ ID NO: 183 - DNA, 15 bp, Artificial Sequence
  h443-457-A ASO for hRPS25 mRNA
gtacagctggttgga

SEQ ID NO: 184 - DNA, 15 bp, Artificial Sequence
  h445-459-A ASO for hRPS25 mRNA
atgtacagctggttg

SEQ ID NO: 185 - DNA, 15 bp, Artificial Sequence
  h448-462-A ASO for hRPS25 mRNA
  modified_base (1)..(1): m5c
caaatgtacagctgg

SEQ ID NO: 186 - DNA, 15 bp, Artificial Sequence
  h449-463-A ASO for hRPS25 mRNA
  modified_base (1)..(1): m5c
  modified_base (2)..(2): m5c
  modified_base (13)..(13): m5c
ccaaatgtacagctg

SEQ ID NO: 187 - DNA, 15 bp, Artificial Sequence
  h450-464-A ASO for hRPS25 mRNA
  modified_base (2)..(2): m5c
  modified_base (3)..(3): m5c
  modified_base (14)..(14): m5c
tccaaatgtacagct

SEQ ID NO: 188 - DNA, 15 bp, Artificial Sequence
  h452-466-A ASO for hRPS25 mRNA
  modified_base (13)..(13): m5c
tttccaaatgtacag

SEQ ID NO: 189 - DNA, 15 bp, Artificial Sequence
  h453-467-A ASO for hRPS25 mRNA
  modified_base (14)..(14): m5c
ttttccaaatgtaca

SEQ ID NO: 190 - DNA, 15 bp, Artificial Sequence
  h454-468-A ASO for hRPS25 mRNA
tttttccaaatgtac

SEQ ID NO: 191 - DNA, 15 bp, Artificial Sequence
  h455-469-A ASO for hRPS25 mRNA
atttttccaaatgta

SEQ ID NO: 192 - DNA, 15 bp, Artificial Sequence
  hp1-15-A ASO for hRPS25 pre-mRNA
  modified_base (1)..(1): m5c
cggacaaaaaggaag

SEQ ID NO: 193 - DNA, 15 bp, Artificial Sequence
  hp72-86-A ASO for hRPS25 pre-mRNA
  modified_base (3)..(3): m5c
ttcacacccctgaag

SEQ ID NO: 194 - DNA, 15 bp, Artificial Sequence
  hp73-87-A ASO for hRPS25 pre-mRNA
  modified_base (1)..(1): m5c
cttcacacccctgaa

SEQ ID NO: 195 - DNA, 15 bp, Artificial Sequence
  hp74-88-A ASO for hRPS25 pre-mRNA
  modified_base (2)..(2): m5c
acttcacacccctga

SEQ ID NO: 196 - DNA, 15 bp, Artificial Sequence
  hp75-89-A ASO for hRPS25 pre-mRNA
  modified_base (3)..(3): m5c
  modified_base (13)..(13): m5c
gacttcacacccctg

SEQ ID NO: 197 - DNA, 15 bp, Artificial Sequence
  hp76-90-A ASO for hRPS25 pre-mRNA
  modified_base (1)..(1): m5c
  modified_base (13)..(13): m5c
  modified_base (14)..(14): m5c
cgacttcacacccct

SEQ ID NO: 198 - DNA, 15 bp, Artificial Sequence
  hp231-245-A ASO for hRPS25 pre-mRNA
  modified_base (2)..(2): m5c
  modified_base (3)..(3): m5c
  modified_base (14)..(14): m5c
tcccctaatactgcg

SEQ ID NO: 199 - DNA, 15 bp, Artificial Sequence
  hp232-246-A ASO for hRPS25 pre-mRNA
  modified_base (3)..(3): m5c
gtcccctaatactgc

SEQ ID NO: 200 - DNA, 15 bp, Artificial Sequence
  hp233-247-A ASO for hRPS25 pre-mRNA
  modified_base (13)..(13): m5c
agtcccctaatactg

SEQ ID NO: 201 - DNA, 15 bp, Artificial Sequence
  hp261-275-A ASO for hRPS25 pre-mRNA
  modified_base (13)..(13): m5c
  modified_base (14)..(14): m5c
atgcaaccaggtcct

SEQ ID NO: 202 - DNA, 15 bp, Artificial Sequence
  hp262-276-A ASO for hRPS25 pre-mRNA
  modified_base (14)..(14): m5c
aatgcaaccaggtcc

SEQ ID NO: 203 - DNA, 15 bp, Artificial Sequence
  hp278-292-A ASO for hRPS25 pre-mRNA
  modified_base (13)..(13): m5c
gtaggagggcagcgg

SEQ ID NO: 204 - DNA, 15 bp, Artificial Sequence
  hp279-293-A ASO for hRPS25 pre-mRNA
  modified_base (14)..(14): m5c
tgtaggagggcagcg

SEQ ID NO: 205 - DNA, 15 bp, Artificial Sequence
  hp280-294-A ASO for hRPS25 pre-mRNA
  modified_base (1)..(1): m5c
ctgtaggagggcagc

SEQ ID NO: 206 - DNA, 15 bp, Artificial Sequence
  hp390-404-A ASO for hRPS25 pre-mRNA
  modified_base (14)..(14): m5c
ggtcttatttctacc

SEQ ID NO: 207 - DNA, 15 bp, Artificial Sequence
  hp392-406-A ASO for hRPS25 pre-mRNA
  modified_base (13)..(13): m5c
gaggtcttatttcta

SEQ ID NO: 208 - DNA, 15 bp, Artificial Sequence
  hp417-431-A ASO for hRPS25 pre-mRNA
agagttacccctagt

SEQ ID NO: 209 - DNA, 15 bp, Artificial Sequence
  hp418-432-A ASO for hRPS25 pre-mRNA
gagagttacccctag

SEQ ID NO: 210 - DNA, 15 bp, Artificial Sequence
  hp419-433-A ASO for hRPS25 pre-mRNA
  modified_base (13)..(13): m5c
agagagttaccccta

SEQ ID NO: 211 - DNA, 15 bp, Artificial Sequence
  hp420-434-A ASO for hRPS25 pre-mRNA
  modified_base (13)..(13): m5c
  modified_base (14)..(14): m5c
gagagagttacccct

SEQ ID NO: 212 - DNA, 15 bp, Artificial Sequence
  hp421-435-A ASO for hRPS25 pre-mRNA
  modified_base (1)..(1): m5c
  modified_base (13)..(13): m5c
  modified_base (14)..(14): m5c
cgagagagttacccc

SEQ ID NO: 213 - DNA, 15 bp, Artificial Sequence
  hp422-436-A ASO for hRPS25 pre-mRNA
  modified_base (2)..(2): m5c
  modified_base (13)..(13): m5c
  modified_base (14)..(14): m5c
acgagagagttaccc

SEQ ID NO: 214 - DNA, 15 bp, Artificial Sequence
  hp423-437-A ASO for hRPS25 pre-mRNA
  modified_base (3)..(3): m5c
  modified_base (14)..(14): m5c
tacgagagagttacc

SEQ ID NO: 215 - DNA, 15 bp, Artificial Sequence
  hp445-459-A ASO for hRPS25 pre-mRNA
  modified_base (14)..(14): m5c
aagttacctattact

SEQ ID NO: 216 - DNA, 15 bp, Artificial Sequence
  hp446-460-A ASO for hRPS25 pre-mRNA
  modified_base (1)..(1): m5c
caagttacctattac

SEQ ID NO: 217 - DNA, 15 bp, Artificial Sequence
  hp447-461-A ASO for hRPS25 pre-mRNA
  modified_base (2)..(2): m5c
acaagttacctatta

SEQ ID NO: 218 - DNA, 15 bp, Artificial Sequence
  hp448-462-A ASO for hRPS25 pre-mRNA
  modified_base (3)..(3): m5c
tacaagttacctatt

SEQ ID NO: 219 - DNA, 15 bp, Artificial Sequence
  hp458-472-A ASO for hRPS25 pre-mRNA
  modified_base (1)..(1): m5c
  modified_base (2)..(2): m5c
  modified_base (13)..(13): m5c
ccacttactatacaa

SEQ ID NO: 220 - DNA, 15 bp, Artificial Sequence
  hp460-474-A ASO for hRPS25 pre-mRNA
  modified_base (3)..(3): m5c
aaccacttactatac

SEQ ID NO: 221 - DNA, 15 bp, Artificial Sequence
  hp461-475-A ASO for hRPS25 pre-mRNA
aaaccacttactata

SEQ ID NO: 222 - DNA, 15 bp, Artificial Sequence
  hp510-524-A ASO for hRPS25 pre-mRNA
  modified_base (3)..(3): m5c
gacgggaagataaac

SEQ ID NO: 223 - DNA, 15 bp, Artificial Sequence
  hp561-575-A ASO for hRPS25 pre-mRNA
  modified_base (2)..(2): m5c
  modified_base (13)..(13): m5c
  modified_base (14)..(14): m5c
tcgcacaacagaccc

SEQ ID NO: 224 - DNA, 15 bp, Artificial Sequence
  hp562-576-A ASO for hRPS25 pre-mRNA
  modified_base (3)..(3): m5c
  modified_base (14)..(14): m5c
ttcgcacaacagacc

SEQ ID NO: 225 - DNA, 15 bp, Artificial Sequence
  hp589-603-A ASO for hRPS25 pre-mRNA
  modified_base (13)..(13): m5c
taacacagcaggcac

SEQ ID NO: 226 - DNA, 15 bp, Artificial Sequence
  hp605-619-A ASO for hRPS25 pre-mRNA
  modified_base (1)..(1): m5c
ctagatcagttaaaa

SEQ ID NO: 227 - DNA, 15 bp, Artificial Sequence
  hp606-620-A ASO for hRPS25 pre-mRNA
  modified_base (2)..(2): m5c
actagatcagttaaa

SEQ ID NO: 228 - DNA, 15 bp, Artificial Sequence
  hp626-640-A ASO for hRPS25 pre-mRNA
  modified_base (2)..(2): m5c
  modified_base (13)..(13): m5c
tcaaacaggggccga

SEQ ID NO: 229 - DNA, 15 bp, Artificial Sequence
  hp627-641-A ASO for hRPS25 pre-mRNA
  modified_base (3)..(3): m5c
  modified_base (13)..(13): m5c
  modified_base (14)..(14): m5c
ttcaaacaggggccg

SEQ ID NO: 230 - DNA, 15 bp, Artificial Sequence
  hp628-642-A ASO for hRPS25 pre-mRNA
  modified_base (1)..(1): m5c
  modified_base (14)..(14): m5c
cttcaaacaggggcc

SEQ ID NO: 231 - DNA, 15 bp, Artificial Sequence
  hp629-643-A ASO for hRPS25 pre-mRNA
  modified_base (1)..(1): m5c
  modified_base (2)..(2): m5c
ccttcaaacaggggc

SEQ ID NO: 232 - DNA, 15 bp, Artificial Sequence
  hp632-646-A ASO for hRPS25 pre-mRNA
tggccttcaaacagg

SEQ ID NO: 233 - DNA, 15 bp, Artificial Sequence
  hp633-647-A ASO for hRPS25 pre-mRNA
  modified_base (13)..(13): m5c
ttggccttcaaacag

SEQ ID NO: 234 - DNA, 15 bp, Artificial Sequence
  hp634-648-A ASO for hRPS25 pre-mRNA
  modified_base (14)..(14): m5c
tttggccttcaaaca

SEQ ID NO: 235 - DNA, 15 bp, Artificial Sequence
  hp654-668-A ASO for hRPS25 pre-mRNA
aaaaaaaacaccgac

SEQ ID NO: 236 - DNA, 15 bp, Artificial Sequence
  hp681-695-A ASO for hRPS25 pre-mRNA
  modified_base (13)..(13): m5c
aattacacattacta

SEQ ID NO: 237 - DNA, 15 bp, Artificial Sequence
  hp696-710-A ASO for hRPS25 pre-mRNA
  modified_base (1)..(1): m5c
  modified_base (2)..(2): m5c
ccgttatcaaggata

SEQ ID NO: 238 - DNA, 15 bp, Artificial Sequence
  hp697-711-A ASO for hRPS25 pre-mRNA
  modified_base (2)..(2): m5c
  modified_base (3)..(3): m5c
accgttatcaaggat

SEQ ID NO: 239 - DNA, 15 bp, Artificial Sequence
  hp761-775-A ASO for hRPS25 pre-mRNA
gttagtatttctggc

SEQ ID NO: 240 - DNA, 15 bp, Artificial Sequence
  hp762-776-A ASO for hRPS25 pre-mRNA
agttagtatttctgg

SEQ ID NO: 241 - DNA, 15 bp, Artificial Sequence
  hp764-778-A ASO for hRPS25 pre-mRNA
  modified_base (1)..(1): m5c
  modified_base (14)..(14): m5c
caagttagtatttct

SEQ ID NO: 242 - DNA, 15 bp, Artificial Sequence
  hp1034-1048-A ASO for hRPS25 pre-mRNA
atgcttaacatggtc

SEQ ID NO: 243 - DNA, 15 bp, Artificial Sequence
  hp1035-1049-A ASO for hRPS25 pre-mRNA
gatgcttaacatggt

SEQ ID NO: 244 - DNA, 15 bp, Artificial Sequence
  hp1103-1117-A ASO for hRPS25 pre-mRNA
ttactaacagccaat

SEQ ID NO: 245 - DNA, 15 bp, Artificial Sequence
  hp1104-1118-A ASO for hRPS25 pre-mRNA
  modified_base (13)..(13): m5c
attactaacagccaa

SEQ ID NO: 246 - DNA, 15 bp, Artificial Sequence
  hp1105-1119-A ASO for hRPS25 pre-mRNA
  modified_base (1)..(1): m5c
  modified_base (13)..(13): m5c
  modified_base (14)..(14): m5c
cattactaacagcca

SEQ ID NO: 247 - DNA, 15 bp, Artificial Sequence
  hp1106-1120-A ASO for hRPS25 pre-mRNA
  modified_base (2)..(2): m5c
  modified_base (14)..(14): m5c
acattactaacagcc

SEQ ID NO: 248 - DNA, 15 bp, Artificial Sequence
  hp1107-1121-A ASO for hRPS25 pre-mRNA
  modified_base (3)..(3): m5c
tacattactaacagc

SEQ ID NO: 249 - DNA, 15 bp, Artificial Sequence
  hp1108-1122-A ASO for hRPS25 pre-mRNA
  modified_base (13)..(13): m5c
ttacattactaacag

SEQ ID NO: 250 - DNA, 15 bp, Artificial Sequence
  hp1110-1124-A ASO for hRPS25 pre-mRNA
aattacattactaac

SEQ ID NO: 251 - DNA, 15 bp, Artificial Sequence
  hp1128-1142-A ASO for hRPS25 pre-mRNA
  modified_base (2)..(2): m5c
  modified_base (13)..(13): m5c
tcaggagtaagacgt

SEQ ID NO: 252 - DNA, 15 bp, Artificial Sequence
  hp1129-1143-A ASO for hRPS25 pre-mRNA
  modified_base (3)..(3): m5c
  modified_base (14)..(14): m5c
atcaggagtaagacg

SEQ ID NO: 253 - DNA, 15 bp, Artificial Sequence
  hp1196-1210-A ASO for hRPS25 pre-mRNA
  modified_base (2)..(2): m5c
gcttcactaaactgc

SEQ ID NO: 254 - DNA, 15 bp, Artificial Sequence
  hp1197-1211-A ASO for hRPS25 pre-mRNA
  modified_base (3)..(3): m5c
  modified_base (13)..(13): m5c
ggcttcactaaactg

SEQ ID NO: 255 - DNA, 15 bp, Artificial Sequence
  hp1217-1231-A ASO for hRPS25 pre-mRNA
  modified_base (1)..(1): m5c
cgaaacataaaagat

SEQ ID NO: 256 - DNA, 15 bp, Artificial Sequence
  hp1218-1232-A ASO for hRPS25 pre-mRNA
  modified_base (2)..(2): m5c
tcgaaacataaaaga

SEQ ID NO: 257 - DNA, 15 bp, Artificial Sequence
  hp1219-1233-A ASO for hRPS25 pre-mRNA
  modified_base (1)..(1): m5c
  modified_base (3)..(3): m5c
ctcgaaacataaaag

SEQ ID NO: 258 - DNA, 15 bp, Artificial Sequence
  hp1398-1412-A ASO for hRPS25 pre-mRNA
gtggaattatggtaa

SEQ ID NO: 259 - DNA, 15 bp, Artificial Sequence
  hp1399-1413-A ASO for hRPS25 pre-mRNA
tgtggaattatggta

SEQ ID NO: 260 - DNA, 15 bp, Artificial Sequence
  hp1402-1416-A ASO for hRPS25 pre-mRNA
tattgtggaattatg

SEQ ID NO: 261 - DNA, 15 bp, Artificial Sequence
  hp1408-1422-A ASO for hRPS25 pre-mRNA
  modified_base (1)..(1): m5c
  modified_base (2)..(2): m5c
ccttattattgtgga

SEQ ID NO: 262 - DNA, 15 bp, Artificial Sequence
  hp1409-1423-A ASO for hRPS25 pre-mRNA
  modified_base (2)..(2): m5c
  modified_base (3)..(3): m5c
gccttattattgtgg

SEQ ID NO: 263 - DNA, 15 bp, Artificial Sequence
  hp1410-1424-A ASO for hRPS25 pre-mRNA
  modified_base (3)..(3): m5c
agccttattattgtg

SEQ ID NO: 264 - DNA, 15 bp, Artificial Sequence
  hp1411-1425-A ASO for hRPS25 pre-mRNA
gagccttattattgt

SEQ ID NO: 265 - DNA, 15 bp, Artificial Sequence
  hp1412-1426-A ASO for hRPS25 pre-mRNA
tgagccttattattg

SEQ ID NO: 266 - DNA, 15 bp, Artificial Sequence
  hp1478-1492-A ASO for hRPS25 pre-mRNA
  modified_base (1)..(1): m5c
  modified_base (13)..(13): m5c
cgttgattcacccgc

SEQ ID NO: 267 - DNA, 15 bp, Artificial Sequence
  hp1480-1494-A ASO for hRPS25 pre-mRNA
  modified_base (2)..(2): m5c
  modified_base (3)..(3): m5c
  modified_base (13)..(13): m5c
  modified_base (14)..(14): m5c
tccgttgattcaccc

SEQ ID NO: 268 - DNA, 15 bp, Artificial Sequence
  hp1715-1729-A ASO for hRPS25 pre-mRNA
  modified_base (2)..(2): m5c
  modified_base (14)..(14): m5c
gctccattatcttcc

SEQ ID NO: 269 - DNA, 15 bp, Artificial Sequence
  hp1749-1763-A ASO for hRPS25 pre-mRNA
  modified_base (1)..(1): m5c
  modified_base (13)..(13): m5c
cgatcatctatcctt

SEQ ID NO: 270 - DNA, 15 bp, Artificial Sequence
  hp1750-1764-A ASO for hRPS25 pre-mRNA
  modified_base (2)..(2): m5c
  modified_base (13)..(13): m5c
  modified_base (14)..(14): m5c
acgatcatctatcct

SEQ ID NO: 271 - DNA, 15 bp, Artificial Sequence
  hp1751-1765-A ASO for hRPS25 pre-mRNA
  modified_base (3)..(3): m5c
  modified_base (14)..(14): m5c
aacgatcatctatcc

SEQ ID NO: 272 - DNA, 15 bp, Artificial Sequence
  hp1763-1777-A ASO for hRPS25 pre-mRNA
  modified_base (3)..(3): m5c
atcctagtttttaac

SEQ ID NO: 273 - DNA, 15 bp, Artificial Sequence
  hp1793-1807-A ASO for hRPS25 pre-mRNA
attgcttaatctgac

SEQ ID NO: 274 - DNA, 15 bp, Artificial Sequence
  hp1885-1899-A ASO for hRPS25 pre-mRNA
  modified_base (13)..(13): m5c
atggtcttaaaactc

SEQ ID NO: 275 - DNA, 15 bp, Artificial Sequence
  hp1887-1901-A ASO for hRPS25 pre-mRNA
gaatggtcttaaaac

SEQ ID NO: 276 - DNA, 15 bp, Artificial Sequence
  hp2047-2061-A ASO for hRPS25 pre-mRNA
  modified_base (13)..(13): m5c
gtttgttttggccgg

SEQ ID NO: 277 - DNA, 15 bp, Artificial Sequence
  hp2048-2062-A ASO for hRPS25 pre-mRNA
  modified_base (13)..(13): m5c
  modified_base (14)..(14): m5c
ggtttgttttggccg

SEQ ID NO: 278 - DNA, 15 bp, Artificial Sequence
  hp2049-2063-A ASO for hRPS25 pre-mRNA
  modified_base (14)..(14): m5c
aggtttgttttggcc

SEQ ID NO: 279 - DNA, 15 bp, Artificial Sequence
  hp2121-2135-A ASO for hRPS25 pre-mRNA
  modified_base (14)..(14): m5c
gaattggtggttgca

SEQ ID NO: 280 - DNA, 15 bp, Artificial Sequence
  hp2122-2136-A ASO for hRPS25 pre-mRNA
ggaattggtggttgc

SEQ ID NO: 281 - DNA, 15 bp, Artificial Sequence
  hp2123-2137-A ASO for hRPS25 pre-mRNA
aggaattggtggttg

SEQ ID NO: 282 - DNA, 15 bp, Artificial Sequence
  hp2124-2138-A ASO for hRPS25 pre-mRNA
  modified_base (1)..(1): m5c
caggaattggtggtt

SEQ ID NO: 283 - DNA, 15 bp, Artificial Sequence
  hp2260-2274-A ASO for hRPS25 pre-mRNA
  modified_base (13)..(13): m5c
ggtaaggagttgcac

SEQ ID NO: 284 - DNA, 15 bp, Artificial Sequence
  hp2261-2275-A ASO for hRPS25 pre-mRNA
  modified_base (14)..(14): m5c
aggtaaggagttgca

SEQ ID NO: 285 - DNA, 15 bp, Artificial Sequence
  hp2262-2276-A ASO for hRPS25 pre-mRNA
gaggtaaggagttgc

SEQ ID NO: 286 - DNA, 15 bp, Artificial Sequence
  hp2268-2282-A ASO for hRPS25 pre-mRNA
tagcttgaggtaagg

SEQ ID NO: 287 - DNA, 15 bp, Artificial Sequence
  hp2269-2283-A ASO for hRPS25 pre-mRNA
atagcttgaggtaag

SEQ ID NO: 288 - DNA, 15 bp, Artificial Sequence
  hp2271-2285-A ASO for hRPS25 pre-mRNA
agatagcttgaggta

SEQ ID NO: 289 - DNA, 15 bp, Artificial Sequence
  hp2277-2291-A ASO for hRPS25 pre-mRNA
  modified_base (2)..(2): m5c
  modified_base (13)..(13): m5c
acgggcagatagctt

SEQ ID NO: 290 - DNA, 15 bp, Artificial Sequence
  hp2339-2353-A ASO for hRPS25 pre-mRNA
  modified_base (14)..(14): m5c
gtaaggtttttggct

SEQ ID NO: 291 - DNA, 15 bp, Artificial Sequence
  hp2341-2355-A ASO for hRPS25 pre-mRNA
tagtaaggtttttgg

SEQ ID NO: 292 - DNA, 15 bp, Artificial Sequence
  hp2342-2356-A ASO for hRPS25 pre-mRNA
  modified_base (1)..(1): m5c
ctagtaaggtttttg

SEQ ID NO: 293 - DNA, 15 bp, Artificial Sequence
  hp2386-2400-A ASO for hRPS25 pre-mRNA
agagaatagcacgat

SEQ ID NO: 294 - DNA, 15 bp, Artificial Sequence
  hp2406-2420-A ASO for hRPS25 pre-mRNA
  modified_base (13)..(13): m5c
gtttgataagtccta

SEQ ID NO: 295 - DNA, 15 bp, Artificial Sequence
  hp2538-2552-A ASO for hRPS25 pre-mRNA
  modified_base (14)..(14): m5c
tttgtatctacctcc

SEQ ID NO: 296 - DNA, 15 bp, Artificial Sequence
  hp2540-2554-A ASO for hRPS25 pre-mRNA
  modified_base (2)..(2): m5c
  modified_base (13)..(13): m5c
  modified_base (14)..(14): m5c
gctttgtatctacct

SEQ ID NO: 297 - DNA, 15 bp, Artificial Sequence
  hp2541-2555-A ASO for hRPS25 pre-mRNA
  modified_base (3)..(3): m5c
  modified_base (14)..(14): m5c
agctttgtatctacc

SEQ ID NO: 298 - DNA, 15 bp, Artificial Sequence
  hp2585-2599-A ASO for hRPS25 pre-mRNA
  modified_base (1)..(1): m5c
ctggttggacctgta

SEQ ID NO: 299 - DNA, 15 bp, Artificial Sequence
  hp2586-2600-A ASO for hRPS25 pre-mRNA
  modified_base (2)..(2): m5c
gctggttggacctgt

SEQ ID NO: 300 - DNA, 15 bp, Artificial Sequence
  hp2587-2601-A ASO for hRPS25 pre-mRNA
  modified_base (3)..(3): m5c
  modified_base (13)..(13): m5c
agctggttggacctg

SEQ ID NO: 301 - DNA, 15 bp, Artificial Sequence
  hp2583-2597-A ASO for hRPS25 pre-mRNA
ggttggacctgtaaa

SEQ ID NO: 302 - DNA, 15 bp, Artificial Sequence
  hp2584-2598-A ASO for hRPS25 pre-mRNA
tggttggacctgtaa

SEQ ID NO: 303 - DNA, 16 bp, Artificial Sequence
  h125-140-A ASO for hRPS25 mRNA
  modified_base (1)..(2): m5c
  modified_base (15)..(15): m5c
cccggatttgttcact

SEQ ID NO: 304 - DNA, 16 bp, Artificial Sequence
  h125-140-B ASO for hRPS25 mRNA
  modified_base (1)..(3): m5c
  modified_base (15)..(15): m5c
cccggatttgttcact

SEQ ID NO: 305 - DNA, 17 bp, Artificial Sequence
  h124-140-C ASO for hRPS25 mRNA
  modified_base (1)..(2): m5c
  modified_base (15)..(15): m5c
cccggatttgttcactg

SEQ ID NO: 306 - DNA, 15 bp, Artificial Sequence
  h187-201-D ASO for hRPS25 mRNA
  modified_base (1)..(1): m5c
  modified_base (14)..(14): m5c
ctaagttattgagct

SEQ ID NO: 307 - DNA, 15 bp, Artificial Sequence
  h187-201-E ASO for hRPS25 mRNA
  modified_base (1)..(1): m5c
  modified_base (14)..(14): m5c
ctaagttattgagct

SEQ ID NO: 308 - DNA, 16 bp, Artificial Sequence
  h186-201-A ASO for hRPS25 mRNA
  modified_base (1)..(1): m5c
ctaagttattgagctt

SEQ ID NO: 309 - DNA, 17 bp, Artificial Sequence
  h186-202-A1 ASO for hRPS25 mRNA
  modified_base (2)..(2): m5c
actaagttattgagctt

SEQ ID NO: 310 - DNA, 17 bp, Artificial Sequence
  h186-202-B1 ASO for hRPS25 mRNA
  modified_base (2)..(2): m5c
  modified_base (15)..(15): m5c
actaagttattgagctt

SEQ ID NO: 311 - DNA, 17 bp, Artificial Sequence
  h186-202-C ASO for hRPS25 mRNA
  modified_base (2)..(2): m5c
  modified_base (15)..(15): m5c
actaagttattgagctt

SEQ ID NO: 312 - DNA, 18 bp, Artificial Sequence
  h186-203-A ASO for hRPS25 mRNA
  modified_base (16)..(16): m5c
gactaagttattgagctt

SEQ ID NO: 313 - DNA, 15 bp, Artificial Sequence
  h214-228-B ASO for hRPS25 mRNA
  modified_base (13)..(13): m5c
tatcataggtagctt

SEQ ID NO: 314 - DNA, 16 bp, Artificial Sequence
  h213-228-A ASO for hRPS25 mRNA
  modified_base (4)..(4): m5c
taucataggtagcttt

SEQ ID NO: 315 - DNA, 16 bp, Artificial Sequence
  h214-229-A ASO for hRPS25 mRNA
  modified_base (14)..(14): m5c
ttatcataggtagctt

SEQ ID NO: 316 - DNA, 15 bp, Artificial Sequence
  h259-273-B ASO for hRPS25 mRNA
  modified_base (1)..(1): m5c
cagctggggttataa

SEQ ID NO: 317 - DNA, 15 bp, Artificial Sequence
  h265-279-A ASO for hRPS25 mRNA
agaccacagctgggg

SEQ ID NO: 318 - DNA, 15 bp, Artificial Sequence
  h266-280-A ASO for hRPS25 mRNA
gagaccacagctggg

SEQ ID NO: 319 - DNA, 15 bp, Artificial Sequence
  h267-281-A ASO for hRPS25 mRNA
agagaccacagctgg

SEQ ID NO: 320 - DNA, 15 bp, Artificial Sequence
  h268-282-A ASO for hRPS25 mRNA
  modified_base (1)..(1): m5c
  modified_base (13)..(13): m5c
cagagaccacagctg

SEQ ID NO: 321 - DNA, 16 bp, Artificial Sequence
  h259-274-A ASO for hRPS25 mRNA
  modified_base (2)..(2): m5c
acagctggggttataa

SEQ ID NO: 322 - DNA, 17 bp, Artificial Sequence
  h263-279-A ASO for hRPS25 mRNA
agaccacagctggggtt

SEQ ID NO: 323 - DNA, 17 bp, Artificial Sequence
  h264-280-A ASO for hRPS25 mRNA
gagaccacagctggggt

SEQ ID NO: 324 - DNA, 15 bp, Artificial Sequence
  h295-309-B ASO for hRPS25 mRNA
  modified_base (1)..(2): m5c
ccagggagcctcgaa

SEQ ID NO: 325 - DNA, 15 bp, Artificial Sequence
  h295-309-C ASO for hRPS25 mRNA
  modified_base (1)..(2): m5c
ccagggagcctcgaa

SEQ ID NO: 326 - DNA, 15 bp, Artificial Sequence
  h296-310-B ASO for hRPS25 mRNA
  modified_base (2)..(3): m5c
  modified_base (13)..(13): m5c
gccagggagcctcga

SEQ ID NO: 327 - DNA, 15 bp, Artificial Sequence
  h296-310-C ASO for hRPS25 mRNA
  modified_base (2)..(3): m5c
  modified_base (13)..(13): m5c
gccagggagcctcga

SEQ ID NO: 328 - DNA, 15 bp, Artificial Sequence
  h300-314-B ASO for hRPS25 mRNA
  modified_base (1)..(2): m5c
  modified_base (14)..(15): m5c
cctggccagggagcc

SEQ ID NO: 329 - DNA, 15 bp, Artificial Sequence
  h300-314-C ASO for hRPS25 mRNA
  modified_base (1)..(2): m5c
  modified_base (14)..(15): m5c
cctggccagggagcc

SEQ ID NO: 330 - DNA, 15 bp, Artificial Sequence
  h301-315-A ASO for hRPS25 mRNA
  modified_base (1)..(3): m5c
  modified_base (15)..(15): m5c
ccctggccagggagc

SEQ ID NO: 331 - DNA, 15 bp, Artificial Sequence
  h302-316-A ASO for hRPS25 mRNA
  modified_base (2)..(3): m5c
gccctggccagggag

SEQ ID NO: 332 - DNA, 15 bp, Artificial Sequence
  h303-317-A ASO for hRPS25 mRNA
  modified_base (3)..(3): m5c
tgccctggccaggga

SEQ ID NO: 333 - DNA, 15 bp, Artificial Sequence
  h304-318-A ASO for hRPS25 mRNA
  modified_base (1)..(1): m5c
ctgccctggccaggg

SEQ ID NO: 334 - DNA, 16 bp, Artificial Sequence
  h296-311-A ASO for hRPS25 mRNA
  modified_base (3)..(3): m5c
  modified_base (14)..(14): m5c
ggccagggagcctcga

SEQ ID NO: 335 - DNA, 16 bp, Artificial Sequence
  h296-311-B ASO for hRPS25 mRNA
  modified_base (3)..(3): m5c
  modified_base (14)..(14): m5c
ggccagggagcctcga

SEQ ID NO: 336 - DNA, 17 bp, Artificial Sequence
  h295-311-A ASO for hRPS25 mRNA
  modified_base (3)..(3): m5c
ggccagggagcctcgaa

SEQ ID NO: 337 - DNA, 17 bp, Artificial Sequence
  h300-316-A ASO for hRPS25 mRNA
  modified_base (2)..(3): m5c
  modified_base (16)..(17): m5c
gccctggccagggagcc

SEQ ID NO: 338 - DNA, 15 bp, Artificial Sequence
  h323-337-B ASO for hRPS25 mRNA
  modified_base (1)..(1): m5c
ctaaggagctcctga

SEQ ID NO: 339 - DNA, 15 bp, Artificial Sequence
  h323-337-C ASO for hRPS25 mRNA
  modified_base (1)..(1): m5c
ctaaggagctcctga

SEQ ID NO: 340 - DNA, 15 bp, Artificial Sequence
  h326-340-D ASO for hRPS25 mRNA
  modified_base (14)..(15): m5c
ttactaaggagctcc

SEQ ID NO: 341 - DNA, 15 bp, Artificial Sequence
  h326-340-E ASO for hRPS25 mRNA
  modified_base (14)..(15): m5c
ttactaaggagctcc

SEQ ID NO: 342 - DNA, 16 bp, Artificial Sequence
  h325-340-A ASO for hRPS25 mRNA
  modified_base (15)..(15): m5c
ttactaaggagctcct

SEQ ID NO: 343 - DNA, 16 bp, Artificial Sequence
  h325-340-B ASO for hRPS25 mRNA
  modified_base (14)..(15): m5c
ttactaaggagctcct

SEQ ID NO: 344 - DNA, 16 bp, Artificial Sequence
  h326-341-A ASO for hRPS25 mRNA
  modified_base (15)..(16): m5c
ttuactaaggagctcc

SEQ ID NO: 345 - DNA, 16 bp, Artificial Sequence
  h326-341-B ASO for hRPS25 mRNA
  modified_base (15)..(16): m5c
ttuactaaggagctcc

SEQ ID NO: 346 - DNA, 16 bp, Artificial Sequence
  h326-341-C ASO for hRPS25 mRNA
  modified_base (15)..(16): m5c
tttactaaggagctcc

SEQ ID NO: 347 - DNA, 16 bp, Artificial Sequence
  h326-341-D ASO for hRPS25 mRNA
  modified_base (13)..(13): m5c
  modified_base (15)..(16): m5c
tttactaaggagcucc

SEQ ID NO: 348 - DNA, 16 bp, Artificial Sequence
  h326-341-E ASO for hRPS25 mRNA
  modified_base (13)..(13): m5c
  modified_base (15)..(16): m5c
tttactaaggagcucc

SEQ ID NO: 349 - DNA, 17 bp, Artificial Sequence
  h322-338-A ASO for hRPS25 mRNA
  modified_base (2)..(2): m5c
actaaggagctcctgaa

SEQ ID NO: 350 - DNA, 17 bp, Artificial Sequence
  h322-338-B ASO for hRPS25 mRNA
  modified_base (2)..(2): m5c
actaaggagctcctgaa

SEQ ID NO: 351 - DNA, 17 bp, Artificial Sequence
  h325-341-C ASO for hRPS25 mRNA
  modified_base (15)..(16): m5c
tttactaaggagctcct

SEQ ID NO: 352 - DNA, 17 bp, Artificial Sequence
  h325-341-D ASO for hRPS25 mRNA
  modified_base (15)..(16): m5c
tttactaaggagctcct

SEQ ID NO: 353 - DNA, 17 bp, Artificial Sequence
  h325-341-E ASO for hRPS25 mRNA
  modified_base (15)..(16): m5c
tttactaaggagctcct

SEQ ID NO: 354 - DNA, 17 bp, Artificial Sequence
  h325-341-F ASO for hRPS25 mRNA
  modified_base (15)..(16): m5c
tttactaaggagctcct

SEQ ID NO: 355 - DNA, 17 bp, Artificial Sequence
  h325-341-G ASO for hRPS25 mRNA
  modified_base (15)..(16): m5c
tttactaaggagctcct

SEQ ID NO: 356 - DNA, 15 bp, Artificial Sequence
  h439-453-B ASO for hRPS25 mRNA
  modified_base (3)..(3): m5c
  modified_base (13)..(13): m5c
agctggttggaccta

SEQ ID NO: 357 - DNA, 15 bp, Artificial Sequence
  h440-454-B ASO for hRPS25 mRNA
  modified_base (1)..(1): m5c
  modified_base (13)..(14): m5c
cagctggttggacct

SEQ ID NO: 358 - DNA, 15 bp, Artificial Sequence
  h440-454-C ASO for hRPS25 mRNA
  modified_base (1)..(1): m5c
  modified_base (13)..(14): m5c
cagctggttggacct

SEQ ID NO: 359 - DNA, 15 bp, Artificial Sequence
  h440-454-D ASO for hRPS25 mRNA
  modified_base (1)..(1): m5c
  modified_base (13)..(14): m5c
cagctggttggacct

SEQ ID NO: 360 - DNA, 15 bp, Artificial Sequence
  h440-454-E ASO for hRPS25 mRNA
  modified_base (1)..(1): m5c
  modified_base (13)..(14): m5c
cagctggttggacct

SEQ ID NO: 361 - DNA, 15 bp, Artificial Sequence
  h451-465-D ASO for hRPS25 mRNA
  modified_base (3)..(3): m5c
  modified_base (15)..(15): m5c
ttccaaatgtacagc

SEQ ID NO: 362 - DNA, 15 bp, Artificial Sequence
  h451-465-E ASO for hRPS25 mRNA
  modified_base (3)..(3): m5c
  modified_base (15)..(15): m5c
ttccaaatgtacagc

SEQ ID NO: 363 - DNA, 15 bp, Artificial Sequence
  h451-465-F ASO for hRPS25 mRNA
  modified_base (3)..(3): m5c
  modified_base (15)..(15): m5c
ttccaaatgtacagc

SEQ ID NO: 364 - DNA, 15 bp, Artificial Sequence
  h451-465-G ASO for hRPS25 mRNA
  modified_base (3)..(3): m5c
  modified_base (15)..(15): m5c
ttccaaatgtacagc

SEQ ID NO: 365 - DNA, 15 bp, Artificial Sequence
  h451-465-H ASO for hRPS25 mRNA
  modified_base (3)..(3): m5c
  modified_base (12)..(12): m5c
  modified_base (15)..(15): m5c
ttccaaatgtacagc

SEQ ID NO: 366 - DNA, 16 bp, Artificial Sequence
  h439-454-A ASO for hRPS25 mRNA
  modified_base (1)..(1): m5c
  modified_base (4)..(4): m5c
  modified_base (14)..(14): m5c
cagctggttggaccta

SEQ ID NO: 367 - DNA, 16 bp, Artificial Sequence
  h439-454-B ASO for hRPS25 mRNA
  modified_base (1)..(1): m5c
  modified_base (4)..(4): m5c
  modified_base (14)..(14): m5c
cagctggttggaccta

SEQ ID NO: 368 - DNA, 16 bp, Artificial Sequence
  h439-454-C ASO for hRPS25 mRNA
  modified_base (1)..(1): m5c
  modified_base (4)..(4): m5c
  modified_base (14)..(14): m5c
cagctggttggaccta

SEQ ID NO: 369 - DNA, 16 bp, Artificial Sequence
  h442-457-A ASO for hRPS25 mRNA
  modified_base (16)..(16): m5c
gtacagctggttggac

SEQ ID NO: 370 - DNA, 16 bp, Artificial Sequence
  h442-457-B ASO for hRPS25 mRNA
  modified_base (16)..(16): m5c
gtacagctggttggac

SEQ ID NO: 371 - DNA, 16 bp, Artificial Sequence
  h443-458-A ASO for hRPS25 mRNA
tgtacagctggttgga

SEQ ID NO: 372 - DNA, 16 bp, Artificial Sequence
  h450-465-A ASO for hRPS25 mRNA
  modified_base (3)..(3): m5c
  modified_base (15)..(15): m5c
ttccaaatgtacagct

SEQ ID NO: 373 - DNA, 16 bp, Artificial Sequence
  h450-465-B ASO for hRPS25 mRNA
  modified_base (3)..(3): m5c
  modified_base (15)..(15): m5c
ttccaaatgtacagct

SEQ ID NO: 374 - DNA, 16 bp, Artificial Sequence
  h450-465-C ASO for hRPS25 mRNA
  modified_base (3)..(3): m5c
  modified_base (15)..(15): m5c
ttccaaatgtacagct

SEQ ID NO: 375 - DNA, 16 bp, Artificial Sequence
  h450-465-D ASO for hRPS25 mRNA
  modified_base (3)..(3): m5c
  modified_base (15)..(15): m5c
ttccaaatgtacagct

SEQ ID NO: 376 - DNA, 16 bp, Artificial Sequence
  h451-466-A ASO for hRPS25 mRNA
  modified_base (16)..(16): m5c
tttccaaatgtacagc

SEQ ID NO: 377 - DNA, 16 bp, Artificial Sequence
  h451-466-B ASO for hRPS25 mRNA
  modified_base (13)..(13): m5c
  modified_base (16)..(16): m5c
tttccaaatgtacagc

SEQ ID NO: 378 - DNA, 16 bp, Artificial Sequence
  h451-466-C ASO for hRPS25 mRNA
  modified_base (13)..(13): m5c
  modified_base (16)..(16): m5c
tttccaaatgtacagc

SEQ ID NO: 379 - DNA, 16 bp, Artificial Sequence
  h451-466-D ASO for hRPS25 mRNA
  modified_base (13)..(13): m5c
  modified_base (16)..(16): m5c
tttccaaatgtacagc

SEQ ID NO: 380 - DNA, 16 bp, Artificial Sequence
  h451-466-E ASO for hRPS25 mRNA
  modified_base (13)..(13): m5c
  modified_base (16)..(16): m5c
tttccaaatgtacagc

SEQ ID NO: 381 - DNA, 16 bp, Artificial Sequence
  h451-466-F ASO for hRPS25 mRNA
  modified_base (13)..(13): m5c
  modified_base (16)..(16): m5c
tttccaaatgtacagc

SEQ ID NO: 382 - DNA, 17 bp, Artificial Sequence
  h429-445-A ASO for hRPS25 mRNA
  modified_base (17)..(17): m5c
ggacctattcatgcatc

SEQ ID NO: 383 - DNA, 17 bp, Artificial Sequence
  h430-446-A ASO for hRPS25 mRNA
  modified_base (15)..(15): m5c
tggacctattcatgcat

SEQ ID NO: 384 - DNA, 17 bp, Artificial Sequence
  h434-450-A ASO for hRPS25 mRNA
  modified_base (15)..(15): m5c
tggttggacctattcat

SEQ ID NO: 385 - DNA, 17 bp, Artificial Sequence
  h439-455-A ASO for hRPS25 mRNA
  modified_base (2)..(2): m5c
  modified_base (15)..(15): m5c
acagctggttggaccta

SEQ ID NO: 386 - DNA, 17 bp, Artificial Sequence
  h441-457-A ASO for hRPS25 mRNA
  modified_base (16)..(17): m5c
gtacagctggttggacc

SEQ ID NO: 387 - DNA, 17 bp, Artificial Sequence
  h441-457-B ASO for hRPS25 mRNA
  modified_base (16)..(17): m5c
gtacagctggttggacc

SEQ ID NO: 388 - DNA, 17 bp, Artificial Sequence
  h442-458-C ASO for hRPS25 mRNA
  modified_base (17)..(17): m5c
tgtacagctggttggac

SEQ ID NO: 389 - DNA, 17 bp, Artificial Sequence
  h442-458-D ASO for hRPS25 mRNA
  modified_base (17)..(17): m5c
tgtacagctggttggac

SEQ ID NO: 390 - DNA, 17 bp, Artificial Sequence
  h442-458-E ASO for hRPS25 mRNA
  modified_base (17)..(17): m5c
tgtacagctggttggac

SEQ ID NO: 391 - DNA, 17 bp, Artificial Sequence
  h443-459-A ASO for hRPS25 mRNA
atgtacagctggttgga

SEQ ID NO: 392 - DNA, 17 bp, Artificial Sequence
  h449-465-A ASO for hRPS25 mRNA
  modified_base (3)..(3): m5c
  modified_base (15)..(15): m5c
ttccaaatgtacagctg

SEQ ID NO: 393 - DNA, 17 bp, Artificial Sequence
  h449-465-B ASO for hRPS25 mRNA
  modified_base (3)..(3): m5c
  modified_base (15)..(15): m5c
ttccaaatgtacagctg

SEQ ID NO: 394 - DNA, 17 bp, Artificial Sequence
  h449-465-C ASO for hRPS25 mRNA
  modified_base (3)..(3): m5c
  modified_base (15)..(15): m5c
ttccaaatgtacagctg

SEQ ID NO: 395 - DNA, 17 bp, Artificial Sequence
  h449-465-D ASO for hRPS25 mRNA
  modified_base (3)..(3): m5c
  modified_base (15)..(15): m5c
ttccaaatgtacagctg

SEQ ID NO: 396 - DNA, 17 bp, Artificial Sequence
  h449-465-E ASO for hRPS25 mRNA
  modified_base (3)..(3): m5c
ttccaaatgtacagctg

SEQ ID NO: 397 - DNA, 19 bp, Artificial Sequence
  h449-467-C ASO for hRPS25 mRNA
ttutccaaatgtacagctg

SEQ ID NO: 398 - DNA, 17 bp, Artificial Sequence
  h442-458-F ASO for hRPS25 mRNA
  modified_base (5)..(5): m5c
  modified_base (8)..(8): m5c
  modified_base (17)..(17): m5c
tgtacagctggttggac

SEQ ID NO: 399 - DNA, 19 bp, Artificial Sequence
  h442-460-C ASO for hRPS25 mRNA
  modified_base (7)..(7): m5c
  modified_base (10)..(10): m5c
  modified_base (19)..(19): m5c
aatgtacagctggttggac

SEQ ID NO: 400 - DNA, 18 bp, Artificial Sequence
  h442-459-A ASO for hRPS25 mRNA
  modified_base (6)..(6): m5c
  modified_base (9)..(9): m5c
  modified_base (18)..(18): m5c
atgtacagctggttggac

SEQ ID NO: 401 - DNA, 18 bp, Artificial Sequence
  h442-459-B ASO for hRPS25 mRNA
  modified_base (6)..(6): m5c
  modified_base (9)..(9): m5c
  modified_base (18)..(18): m5c
atgtacagctggttggac

SEQ ID NO: 402 - DNA, 18 bp, Artificial Sequence
  h443-460-A ASO for hRPS25 mRNA
  modified_base (7)..(7): m5c
  modified_base (10)..(10): m5c
aatgtacagctggttgga

SEQ ID NO: 403 - DNA, 18 bp, Artificial Sequence
  h443-460-B ASO for hRPS25 mRNA
  modified_base (7)..(7): m5c
  modified_base (10)..(10): m5c
aatgtacagctggttgga

SEQ ID NO: 404 - DNA, 19 bp, Artificial Sequence
  h447-465-A ASO for hRPS25 mRNA
  modified_base (3)..(4): m5c
  modified_base (12)..(12): m5c
  modified_base (15)..(15): m5c
ttccaaatgtacagctggt

SEQ ID NO: 405 - DNA, 18 bp, Artificial Sequence
  h448-465-A ASO for hRPS25 mRNA
  modified_base (3)..(4): m5c
  modified_base (12)..(12): m5c
  modified_base (15)..(15): m5c
ttccaaatgtacagctgg

SEQ ID NO: 406 - DNA, 18 bp, Artificial Sequence
  h448-465-B ASO for hRPS25 mRNA
  modified_base (3)..(4): m5c
  modified_base (12)..(12): m5c
  modified_base (15)..(15): m5c
ttccaaatgtacagctgg

SEQ ID NO: 407 - DNA, 18 bp, Artificial Sequence
  h449-466-A ASO for hRPS25 mRNA
  modified_base (4)..(5): m5c
  modified_base (13)..(13): m5c
  modified_base (16)..(16): m5c
tttccaaatgtacagctg

SEQ ID NO: 408 - DNA, 18 bp, Artificial Sequence
  h449-466-B ASO for hRPS25 mRNA
  modified_base (4)..(5): m5c
  modified_base (13)..(13): m5c
  modified_base (16)..(16): m5c
tttccaaatgtacagctg

SEQ ID NO: 409 - DNA, 18 bp, Artificial Sequence
  h450-467-A ASO for hRPS25 mRNA
  modified_base (5)..(6): m5c
  modified_base (14)..(14): m5c
  modified_base (17)..(17): m5c
ttttccaaatgtacagct

SEQ ID NO: 410 - DNA, 19 bp, Artificial Sequence
  h448-466-A ASO for hRPS25 mRNA
  modified_base (4)..(5): m5c
  modified_base (13)..(13): m5c
  modified_base (16)..(16): m5c
tttccaaatgtacagctgg

SEQ ID NO: 411 - DNA, 18 bp, Artificial Sequence
  h450-467-B ASO for hRPS25 mRNA
  modified_base (5)..(6): m5c
  modified_base (14)..(14): m5c
  modified_base (17)..(17): m5c
ttttccaaatgtacagct

SEQ ID NO: 412 - DNA, 19 bp, Artificial Sequence
  h450-468-A ASO for hRPS25 mRNA
  modified_base (6)..(7): m5c
  modified_base (15)..(15): m5c
  modified_base (18)..(18): m5c
tttttccaaatgtacagct

SEQ ID NO: 413 - DNA, 17 bp, Artificial Sequence
  h451-467-A ASO for hRPS25 mRNA
  modified_base (5)..(6): m5c
  modified_base (14)..(14): m5c
  modified_base (17)..(17): m5c
ttttccaaatgtacagc

SEQ ID NO: 414 - DNA, 18 bp, Artificial Sequence
  h451-468-A ASO for hRPS25 mRNA
  modified_base (6)..(7): m5c
  modified_base (15)..(15): m5c
  modified_base (18)..(18): m5c
tttttccaaatgtacagc

SEQ ID NO: 415 - DNA, 18 bp, Artificial Sequence
  h451-468-B ASO for hRPS25 mRNA
  modified_base (6)..(7): m5c
  modified_base (15)..(15): m5c
  modified_base (18)..(18): m5c
tttttccaaatgtacagc

SEQ ID NO: 416 - DNA, 19 bp, Artificial Sequence
  h451-469-A ASO for hRPS25 mRNA
  modified_base (7)..(8): m5c
  modified_base (16)..(16): m5c
  modified_base (19)..(19): m5c
atttttccaaatgtacagc

SEQ ID NO: 417 - DNA, 19 bp, Artificial Sequence
  h449-467-D ASO for hRPS25 mRNA
  modified_base (5)..(6): m5c
  modified_base (14)..(14): m5c
  modified_base (17)..(17): m5c
ttttccaaatgtacagctg

SEQ ID NO: 418 - DNA, 15 bp, Artificial Sequence
  h451-465-I ASO for hRPS25 mRNA
  modified_base (3)..(3): m5c
  modified_base (15)..(15): m5c
ttccaaatgtacagc

SEQ ID NO: 419 - DNA, 15 bp, Artificial Sequence
  h451-465-J ASO for hRPS25 mRNA
  modified_base (3)..(3): m5c
  modified_base (15)..(15): m5c
ttccaaatgtacagc

SEQ ID NO: 420 - DNA, 15 bp, Artificial Sequence
  h451-465-K ASO for hRPS25 mRNA
  modified_base (3)..(3): m5c
  modified_base (15)..(15): m5c
ttccaaatgtacagc

SEQ ID NO: 421 - DNA, 15 bp, Artificial Sequence
  h451-465-L ASO for hRPS25 mRNA
  modified_base (3)..(3): m5c
  modified_base (15)..(15): m5c
ttccaaatgtacagc

SEQ ID NO: 422 - DNA, 15 bp, Artificial Sequence
  h451-465-M ASO for hRPS25 mRNA
  modified_base (3)..(3): m5c
  modified_base (15)..(15): m5c
ttccaaatgtacagc

SEQ ID NO: 423 - DNA, 15 bp, Artificial Sequence
  h451-465-N ASO for hRPS25 mRNA
  modified_base (3)..(4): m5c
  modified_base (15)..(15): m5c
ttccaaatgtacagc

SEQ ID NO: 424 - DNA, 15 bp, Artificial Sequence
  h451-465-O ASO for hRPS25 mRNA
  modified_base (3)..(4): m5c
  modified_base (15)..(15): m5c
ttccaaatgtacagc

SEQ ID NO: 425 - DNA, 15 bp, Artificial Sequence
  h451-465-P ASO for hRPS25 mRNA
  modified_base (3)..(3): m5c
  modified_base (15)..(15): m5c
ttccaaatgtacagc

SEQ ID NO: 426 - DNA, 17 bp, Artificial Sequence
  h451-467-B ASO for hRPS25 mRNA
  modified_base (5)..(5): m5c
  modified_base (17)..(17): m5c
ttttccaaatgtacagc

SEQ ID NO: 427 - DNA, 17 bp, Artificial Sequence
  h451-467-C ASO for hRPS25 mRNA
  modified_base (5)..(5): m5c
  modified_base (14)..(14): m5c
  modified_base (17)..(17): m5c
ttttccaaatgtacagc

SEQ ID NO: 428 - DNA, 15 bp, Artificial Sequence
  h451-465-Q ASO for hRPS25 mRNA
  modified_base (3)..(3): m5c
  modified_base (15)..(15): m5c
ttccaaatgtacagc

SEQ ID NO: 429 - DNA, 15 bp, Artificial Sequence
  h451-465-R ASO for hRPS25 mRNA
  modified_base (3)..(3): m5c
  modified_base (15)..(15): m5c
ttccaaatgtacagc

SEQ ID NO: 430 - DNA, 17 bp, Artificial Sequence
  h451-467-D ASO for hRPS25 mRNA
  modified_base (5)..(5): m5c
  modified_base (14)..(14): m5c
  modified_base (17)..(17): m5c
ttttccaaatgtacagc

SEQ ID NO: 431 - DNA, 17 bp, Artificial Sequence
  h451-467-E ASO for hRPS25 mRNA
  modified_base (5)..(5): m5c
  modified_base (17)..(17): m5c
ttttccaaatgtacagc

SEQ ID NO: 432 - DNA, 17 bp, Artificial Sequence
  h451-467-F ASO for hRPS25 mRNA
  modified_base (5)..(5): m5c
  modified_base (14)..(14): m5c
  modified_base (17)..(17): m5c
ttttccaaatgtacagc

SEQ ID NO: 433 - DNA, 17 bp, Artificial Sequence
  h325-341-H ASO for hRPS25 mRNA
  modified_base (15)..(16): m5c
tttactaaggagctcct

SEQ ID NO: 434 - DNA, 17 bp, Artificial Sequence
  h325-341-I ASO for hRPS25 mRNA
  modified_base (5)..(5): m5c
  modified_base (15)..(16): m5c
tttactaaggagctcct

SEQ ID NO: 435 - DNA, 17 bp, Artificial Sequence
  h325-341-J ASO for hRPS25 mRNA
  modified_base (5)..(5): m5c
  modified_base (13)..(13): m5c
  modified_base (15)..(16): m5c
tttactaaggagctcct

SEQ ID NO: 436 - DNA, 17 bp, Artificial Sequence
  h325-341-K ASO for hRPS25 mRNA
  modified_base (5)..(5): m5c
  modified_base (13)..(13): m5c
  modified_base (15)..(16): m5c
tttactaaggagctcct

SEQ ID NO: 437 - DNA, 17 bp, Artificial Sequence
  h325-341-L ASO for hRPS25 mRNA
  modified_base (15)..(16): m5c
tttactaaggagctcct

SEQ ID NO: 438 - DNA, 17 bp, Artificial Sequence
  h325-341-M ASO for hRPS25 mRNA
  modified_base (5)..(5): m5c
  modified_base (15)..(16): m5c
tttactaaggagctcct

SEQ ID NO: 439 - DNA, 17 bp, Artificial Sequence
  h325-341-N ASO for hRPS25 mRNA
  modified_base (15)..(16): m5c
tttactaaggagctcct

SEQ ID NO: 440 - DNA, 17 bp, Artificial Sequence
  h325-341-O ASO for hRPS25 mRNA
  modified_base (15)..(16): m5c
tttactaaggagctcct

SEQ ID NO: 441 - DNA, 17 bp, Artificial Sequence
  h325-341-P ASO for hRPS25 mRNA
  modified_base (15)..(16): m5c
tttactaaggagctcct

SEQ ID NO: 442 - DNA, 17 bp, Artificial Sequence
  h325-341-Q ASO for hRPS25 mRNA
  modified_base (15)..(16): m5c
tttactaaggagctcct

SEQ ID NO: 443 - DNA, 17 bp, Artificial Sequence
  h325-341-R ASO for hRPS25 mRNA
  modified_base (15)..(16): m5c
tttactaaggagctcct

SEQ ID NO: 444 - DNA, 17 bp, Artificial Sequence
  h325-341-S ASO for hRPS25 mRNA
  modified_base (15)..(16): m5c
tttactaaggagctcct

SEQ ID NO: 445 - DNA, 17 bp, Artificial Sequence
  h325-341-T ASO for hRPS25 mRNA
  modified_base (15)..(16): m5c
tttactaaggagctcct

SEQ ID NO: 446 - DNA, 17 bp, Artificial Sequence
  h325-341-U ASO for hRPS25 mRNA
  modified_base (13)..(13): m5c
  modified_base (15)..(16): m5c
tttactaaggagctcct

SEQ ID NO: 447 - DNA, 17 bp, Artificial Sequence
  h325-341-V ASO for hRPS25 mRNA
  modified_base (15)..(16): m5c
tttactaaggagctcct

SEQ ID NO: 448 - DNA, 15 bp, Artificial Sequence
  h451-465-S ASO for hRPS25 mRNA
  modified_base (3)..(4): m5c
  modified_base (15)..(15): m5c
ttccaaatgtacagc

SEQ ID NO: 449 - DNA, 15 bp, Artificial Sequence
  h451-465-T ASO for hRPS25 mRNA
  modified_base (3)..(3): m5c
  modified_base (15)..(15): m5c
ttccaaatgtacagc

SEQ ID NO: 450 - DNA, 15 bp, Artificial Sequence
  h451-465-U ASO for hRPS25 mRNA
  modified_base (3)..(3): m5c
  modified_base (15)..(15): m5c
ttccaaatgtacagc

SEQ ID NO: 451 - DNA, 15 bp, Artificial Sequence
  h451-465-V ASO for hRPS25 mRNA
  modified_base (3)..(3): m5c
  modified_base (15)..(15): m5c
ttccaaatgtacagc

SEQ ID NO: 452 - DNA, 15 bp, Artificial Sequence
  h451-465-W ASO for hRPS25 mRNA
  modified_base (3)..(3): m5c
  modified_base (15)..(15): m5c
ttccaaatgtacagc

SEQ ID NO: 453 - DNA, 15 bp, Artificial Sequence
  h451-465-X ASO for hRPS25 mRNA
  modified_base (3)..(3): m5c
  modified_base (15)..(15): m5c
ttccaaatgtacagc

SEQ ID NO: 454 - DNA, 15 bp, Artificial Sequence
  h451-465-Y ASO for hRPS25 mRNA
  modified_base (3)..(3): m5c
  modified_base (15)..(15): m5c
ttccaaatgtacagc

SEQ ID NO: 455 - DNA, 15 bp, Artificial Sequence
  h451-465-Z ASO for hRPS25 mRNA
  modified_base (3)..(3): m5c
  modified_base (15)..(15): m5c
ttccaaatgtacagc

SEQ ID NO: 456 - DNA, 15 bp, Artificial Sequence
  h451-465-AA ASO for hRPS25 mRNA
  modified_base (3)..(3): m5c
  modified_base (12)..(12): m5c
  modified_base (15)..(15): m5c
ttccaaatgtacagc

SEQ ID NO: 457 - DNA, 15 bp, Artificial Sequence
  h451-465-AB ASO for hRPS25 mRNA
  modified_base (3)..(4): m5c
  modified_base (12)..(12): m5c
  modified_base (15)..(15): m5c
ttccaaatgtacagc

SEQ ID NO: 458 - DNA, 15 bp, Artificial Sequence
  h451-465-AC ASO for hRPS25 mRNA
  modified_base (3)..(4): m5c
  modified_base (12)..(12): m5c
  modified_base (15)..(15): m5c
ttccaaatgtacagc

SEQ ID NO: 459 - DNA, 15 bp, Artificial Sequence
  h451-465-AD ASO for hRPS25 mRNA
  modified_base (3)..(4): m5c
  modified_base (12)..(12): m5c
  modified_base (15)..(15): m5c
ttccaaatgtacagc

SEQ ID NO: 460 - DNA, 15 bp, Artificial Sequence
  h451-465-AE ASO for hRPS25 mRNA
  modified_base (3)..(4): m5c
  modified_base (12)..(12): m5c
  modified_base (15)..(15): m5c
ttccaaatgtacagc

SEQ ID NO: 461 - DNA, 15 bp, Artificial Sequence
  h451-465-AF ASO for hRPS25 mRNA
  modified_base (3)..(4): m5c
  modified_base (12)..(12): m5c
  modified_base (15)..(15): m5c
ttccaaatgtacagc

SEQ ID NO: 462 - DNA, 15 bp, Artificial Sequence
  h451-465-AG ASO for hRPS25 mRNA
  modified_base (3)..(4): m5c
  modified_base (12)..(12): m5c
  modified_base (15)..(15): m5c
ttccaaatgtacagc

SEQ ID NO: 463 - DNA, 15 bp, Artificial Sequence
  h451-465-AH ASO for hRPS25 mRNA
  modified_base (3)..(4): m5c
  modified_base (12)..(12): m5c
  modified_base (15)..(15): m5c
ttccaaatgtacagc

SEQ ID NO: 464 - DNA, 15 bp, Artificial Sequence
  h451-465-AI ASO for hRPS25 mRNA
  modified_base (3)..(4): m5c
  modified_base (12)..(12): m5c
  modified_base (15)..(15): m5c
ttccaaatgtacagc

SEQ ID NO: 465 - DNA, 15 bp, Artificial Sequence
  h451-465-AJ ASO for hRPS25 mRNA
  modified_base (3)..(4): m5c
  modified_base (12)..(12): m5c
  modified_base (15)..(15): m5c
ttccaaatgtacagc

SEQ ID NO: 466 - DNA, 15 bp, Artificial Sequence
  h451-465-AK ASO for hRPS25 mRNA
  modified_base (3)..(4): m5c
  modified_base (12)..(12): m5c
  modified_base (15)..(15): m5c
ttccaaatgtacagc

SEQ ID NO: 467 - DNA, 15 bp, Artificial Sequence
  h451-465-AL ASO for hRPS25 mRNA
  modified_base (3)..(4): m5c
  modified_base (12)..(12): m5c
  modified_base (15)..(15): m5c
ttccaaatgtacagc

SEQ ID NO: 468 - DNA, 15 bp, Artificial Sequence
  h451-465-AM ASO for hRPS25 mRNA
  modified_base (3)..(4): m5c
  modified_base (12)..(12): m5c
  modified_base (15)..(15): m5c
ttccaaatgtacagc

SEQ ID NO: 469 - DNA, 15 bp, Artificial Sequence
  h451-465-AN ASO for hRPS25 mRNA
  modified_base (3)..(3): m5c
  modified_base (15)..(15): m5c
ttcactgacataagc

SEQ ID NO: 470 - DNA, 15 bp, Artificial Sequence
  h451-465-AO ASO for hRPS25 mRNA
  modified_base (3)..(3): m5c
  modified_base (15)..(15): m5c
ttcattgacacaagc

SEQ ID NO: 471 - DNA, 15 bp, Artificial Sequence
  h8-22 ASO for hRPS25 mRNA
cgtcaagatgtcgga

SEQ ID NO: 472 - DNA, 15 bp, Artificial Sequence
  h9-23 ASO for hRPS25 mRNA
tcgtcaagatgtcgg

SEQ ID NO: 473 - DNA, 15 bp, Artificial Sequence
  h10-24 ASO for hRPS25 mRNA
ctcgtcaagatgtcg

SEQ ID NO: 474 - DNA, 15 bp, Artificial Sequence
  h27-41 ASO for hRPS25 mRNA
gcagcagacaccgca

SEQ ID NO: 475 - DNA, 15 bp, Artificial Sequence
  h28-42 ASO for hRPS25 mRNA
agcagcagacaccgc

SEQ ID NO: 476 - DNA, 15 bp, Artificial Sequence
  h29-43 ASO for hRPS25 mRNA
tagcagcagacaccg

SEQ ID NO: 477 - DNA, 15 bp, Artificial Sequence
  h30-44 ASO for hRPS25 mRNA
atagcagcagacacc

SEQ ID NO: 478 - DNA, 15 bp, Artificial Sequence
  h32-46 ASO for hRPS25 mRNA
gaatagcagcagaca

SEQ ID NO: 479 - DNA, 15 bp, Artificial Sequence
  h33-47 ASO for hRPS25 mRNA
agaatagcagcagac

SEQ ID NO: 480 - DNA, 15 bp, Artificial Sequence
  h34-48 ASO for hRPS25 mRNA
gagaatagcagcaga

SEQ ID NO: 481 - DNA, 15 bp, Artificial Sequence
  h35-49 ASO for hRPS25 mRNA
ggagaatagcagcag

SEQ ID NO: 482 - DNA, 15 bp, Artificial Sequence
  h36-50 ASO for hRPS25 mRNA
cggagaatagcagca

SEQ ID NO: 483 - DNA, 15 bp, Artificial Sequence
  h37-51 ASO for hRPS25 mRNA
tcggagaatagcagc

SEQ ID NO: 484 - DNA, 15 bp, Artificial Sequence
  h38-52 ASO for hRPS25 mRNA
ctcggagaatagcag

SEQ ID NO: 485 - DNA, 15 bp, Artificial Sequence
  h39-53 ASO for hRPS25 mRNA
gctcggagaatagca

SEQ ID NO: 486 - DNA, 15 bp, Artificial Sequence
  h40-54 ASO for hRPS25 mRNA
agctcggagaatagc

SEQ ID NO: 487 - DNA, 15 bp, Artificial Sequence
  h72-86 ASO for hRPS25 mRNA
cttcttcttgtcgtc

SEQ ID NO: 488 - DNA, 15 bp, Artificial Sequence
  h79-93 ASO for hRPS25 mRNA
cgtccttcttcttct

SEQ ID NO: 489 - DNA, 15 bp, Artificial Sequence
  h98-112 ASO for hRPS25 mRNA
ttcttggccgacttt

SEQ ID NO: 490 - DNA, 15 bp, Artificial Sequence
  h99-113 ASO for hRPS25 mRNA
tttcttggccgactt

SEQ ID NO: 491 - DNA, 15 bp, Artificial Sequence
  h100-114 ASO for hRPS25 mRNA
ctttcttggccgact

SEQ ID NO: 492 - DNA, 15 bp, Artificial Sequence
  h101-115 ASO for hRPS25 mRNA
tctttcttggccgac

SEQ ID NO: 493 - DNA, 15 bp, Artificial Sequence
  h102-116 ASO for hRPS25 mRNA
gtctttcttggccga

SEQ ID NO: 494 - DNA, 15 bp, Artificial Sequence
  h103-117 ASO for hRPS25 mRNA
tgtctttcttggccg

SEQ ID NO: 495 - DNA, 15 bp, Artificial Sequence
  h104-118 ASO for hRPS25 mRNA
ttgtctttcttggcc

SEQ ID NO: 496 - DNA, 15 bp, Artificial Sequence
  h105-119 ASO for hRPS25 mRNA
tttgtctttcttggc

SEQ ID NO: 497 - DNA, 15 bp, Artificial Sequence
  h106-120 ASO for hRPS25 mRNA
ctttgtctttcttgg

SEQ ID NO: 498 - DNA, 15 bp, Artificial Sequence
  h107-121 ASO for hRPS25 mRNA
tctttgtctttcttg

SEQ ID NO: 499 - DNA, 15 bp, Artificial Sequence
  h122-136 ASO for hRPS25 mRNA
gatttgttcactggg

SEQ ID NO: 500 - DNA, 15 bp, Artificial Sequence
  h123-137 ASO for hRPS25 mRNA
ggatttgttcactgg

SEQ ID NO: 501 - DNA, 15 bp, Artificial Sequence
  h124-138 ASO for hRPS25 mRNA
cggatttgttcactg

SEQ ID NO: 502 - DNA, 15 bp, Artificial Sequence
  h125-139 ASO for hRPS25 mRNA
ccggatttgttcact

SEQ ID NO: 503 - DNA, 15 bp, Artificial Sequence
  h126-140 ASO for hRPS25 mRNA
cccggatttgttcac

SEQ ID NO: 504 - DNA, 15 bp, Artificial Sequence
  h127-141 ASO for hRPS25 mRNA
ccccggatttgttca

SEQ ID NO: 505 - DNA, 15 bp, Artificial Sequence
  h128-142 ASO for hRPS25 mRNA
cccccggatttgttc

SEQ ID NO: 506 - DNA, 15 bp, Artificial Sequence
  h129-143 ASO for hRPS25 mRNA
gcccccggatttgtt

SEQ ID NO: 507 - DNA, 15 bp, Artificial Sequence
  h130-144 ASO for hRPS25 mRNA
tgcccccggatttgt

SEQ ID NO: 508 - DNA, 15 bp, Artificial Sequence
  h140-154 ASO for hRPS25 mRNA
tttttggccttgccc

SEQ ID NO: 509 - DNA, 15 bp, Artificial Sequence
  h160-174 ASO for hRPS25 mRNA
tgcctttggaccact

SEQ ID NO: 510 - DNA, 15 bp, Artificial Sequence
  h161-175 ASO for hRPS25 mRNA
ttgcctttggaccac

SEQ ID NO: 511 - DNA, 15 bp, Artificial Sequence
  h180-194 ASO for hRPS25 mRNA
attgagcttgtcccg

SEQ ID NO: 512 - DNA, 15 bp, Artificial Sequence
  h181-195 ASO for hRPS25 mRNA
tattgagcttgtccc

SEQ ID NO: 513 - DNA, 15 bp, Artificial Sequence
  h182-196 ASO for hRPS25 mRNA
ttattgagcttgtcc

SEQ ID NO: 514 - DNA, 15 bp, Artificial Sequence
  h183-197 ASO for hRPS25 mRNA
gttattgagcttgtc

SEQ ID NO: 515 - DNA, 15 bp, Artificial Sequence
  h184-198 ASO for hRPS25 mRNA
agttattgagcttgt

SEQ ID NO: 516 - DNA, 15 bp, Artificial Sequence
  h185-199 ASO for hRPS25 mRNA
aagttattgagcttg

SEQ ID NO: 517 - DNA, 15 bp, Artificial Sequence
  h186-200 ASO for hRPS25 mRNA
taagttattgagctt

SEQ ID NO: 518 - DNA, 15 bp, Artificial Sequence
  h187-201 ASO for hRPS25 mRNA
ctaagttattgagct

SEQ ID NO: 519 - DNA, 15 bp, Artificial Sequence
  h188-202 ASO for hRPS25 mRNA
actaagttattgagc

SEQ ID NO: 520 - DNA, 15 bp, Artificial Sequence
  h189-203 ASO for hRPS25 mRNA
gactaagttattgag

SEQ ID NO: 521 - DNA, 15 bp, Artificial Sequence
  h190-204 ASO for hRPS25 mRNA
agactaagttattga

SEQ ID NO: 522 - DNA, 15 bp, Artificial Sequence
  h191-205 ASO for hRPS25 mRNA
aagactaagttattg

SEQ ID NO: 523 - DNA, 15 bp, Artificial Sequence
  h193-207 ASO for hRPS25 mRNA
acaagactaagttat

SEQ ID NO: 524 - DNA, 15 bp, Artificial Sequence
  h196-210 ASO for hRPS25 mRNA
caaacaagactaagt

SEQ ID NO: 525 - DNA, 15 bp, Artificial Sequence
  h197-211 ASO for hRPS25 mRNA
tcaaacaagactaag

SEQ ID NO: 526 - DNA, 15 bp, Artificial Sequence
  h208-222 ASO for hRPS25 mRNA
aggtagctttgtcaa

SEQ ID NO: 527 - DNA, 15 bp, Artificial Sequence
  h209-223 ASO for hRPS25 mRNA
taggtagctttgtca

SEQ ID NO: 528 - DNA, 15 bp, Artificial Sequence
  h210-224 ASO for hRPS25 mRNA
ataggtagctttgtc

SEQ ID NO: 529 - DNA, 15 bp, Artificial Sequence
  h211-225 ASO for hRPS25 mRNA
cataggtagctttgt

SEQ ID NO: 530 - DNA, 15 bp, Artificial Sequence
  h212-226 ASO for hRPS25 mRNA
tcataggtagctttg

SEQ ID NO: 531 - DNA, 15 bp, Artificial Sequence
  h213-227 ASO for hRPS25 mRNA
atcataggtagcttt

SEQ ID NO: 532 - DNA, 15 bp, Artificial Sequence
  h214-228 ASO for hRPS25 mRNA
tatcataggtagctt

SEQ ID NO: 533 - DNA, 15 bp, Artificial Sequence
  h215-229 ASO for hRPS25 mRNA
ttatcataggtagct

SEQ ID NO: 534 - DNA, 15 bp, Artificial Sequence
  h216-230 ASO for hRPS25 mRNA
tttatcataggtagc

SEQ ID NO: 535 - DNA, 15 bp, Artificial Sequence
  h217-231 ASO for hRPS25 mRNA
gtttatcataggtag

SEQ ID NO: 536 - DNA, 15 bp, Artificial Sequence
  h218-232 ASO for hRPS25 mRNA
agtttatcataggta

SEQ ID NO: 537 - DNA, 15 bp, Artificial Sequence
  h219-233 ASO for hRPS25 mRNA
gagtttatcataggt

SEQ ID NO: 538 - DNA, 15 bp, Artificial Sequence
  h220-234 ASO for hRPS25 mRNA
agagtttatcatagg

SEQ ID NO: 539 - DNA, 15 bp, Artificial Sequence
  h221-235 ASO for hRPS25 mRNA
cagagtttatcatag

SEQ ID NO: 540 - DNA, 15 bp, Artificial Sequence
  h222-236 ASO for hRPS25 mRNA
acagagtttatcata

SEQ ID NO: 541 - DNA, 15 bp, Artificial Sequence
  h223-237 ASO for hRPS25 mRNA
tacagagtttatcat

SEQ ID NO: 542 - DNA, 15 bp, Artificial Sequence
  h224-238 ASO for hRPS25 mRNA
ttacagagtttatca

SEQ ID NO: 543 - DNA, 15 bp, Artificial Sequence
  h242-256 ASO for hRPS25 mRNA
ttatagttgggaact

SEQ ID NO: 544 - DNA, 15 bp, Artificial Sequence
  h243-257 ASO for hRPS25 mRNA
tttatagttgggaac

SEQ ID NO: 545 - DNA, 15 bp, Artificial Sequence
  h253-267 ASO for hRPS25 mRNA
gggttataagtttat

SEQ ID NO: 546 - DNA, 15 bp, Artificial Sequence
  h254-268 ASO for hRPS25 mRNA
ggggttataagttta

SEQ ID NO: 547 - DNA, 15 bp, Artificial Sequence
  h255-269 ASO for hRPS25 mRNA
tggggttataagttt

SEQ ID NO: 548 - DNA, 15 bp, Artificial Sequence
  h256-270 ASO for hRPS25 mRNA
ctggggttataagtt

SEQ ID NO: 549 - DNA, 15 bp, Artificial Sequence
  h257-271 ASO for hRPS25 mRNA
gctggggttataagt

SEQ ID NO: 550 - DNA, 15 bp, Artificial Sequence
  h258-272 ASO for hRPS25 mRNA
agctggggttataag

SEQ ID NO: 551 - DNA, 15 bp, Artificial Sequence
  h259-273 ASO for hRPS25 mRNA
cagctggggttataa

SEQ ID NO: 552 - DNA, 15 bp, Artificial Sequence
  h260-274 ASO for hRPS25 mRNA
acagctggggttata

SEQ ID NO: 553 - DNA, 15 bp, Artificial Sequence
  h261-275 ASO for hRPS25 mRNA
cacagctggggttat

SEQ ID NO: 554 - DNA, 15 bp, Artificial Sequence
  h262-276 ASO for hRPS25 mRNA
ccacagctggggtta

SEQ ID NO: 555 - DNA, 15 bp, Artificial Sequence
  h263-277 ASO for hRPS25 mRNA
accacagctggggtt

SEQ ID NO: 556 - DNA, 15 bp, Artificial Sequence
  h264-278 ASO for hRPS25 mRNA
gaccacagctggggt

SEQ ID NO: 557 - DNA, 15 bp, Artificial Sequence
  h285-299 ASO for hRPS25 mRNA
tcgaatcttcagtct

SEQ ID NO: 558 - DNA, 15 bp, Artificial Sequence
  h286-300 ASO for hRPS25 mRNA
ctcgaatcttcagtc

SEQ ID NO: 559 - DNA, 15 bp, Artificial Sequence
  h291-305 ASO for hRPS25 mRNA
ggagcctcgaatctt

SEQ ID NO: 560 - DNA, 15 bp, Artificial Sequence
  h292-306 ASO for hRPS25 mRNA
gggagcctcgaatct

SEQ ID NO: 561 - DNA, 15 bp, Artificial Sequence
  h293-307 ASO for hRPS25 mRNA
agggagcctcgaatc

SEQ ID NO: 562 - DNA, 15 bp, Artificial Sequence
  h294-308 ASO for hRPS25 mRNA
cagggagcctcgaat

SEQ ID NO: 563 - DNA, 15 bp, Artificial Sequence
  h295-309 ASO for hRPS25 mRNA
ccagggagcctcgaa

SEQ ID NO: 564 - DNA, 15 bp, Artificial Sequence
  h296-310 ASO for hRPS25 mRNA
gccagggagcctcga

SEQ ID NO: 565 - DNA, 15 bp, Artificial Sequence
  h297-311 ASO for hRPS25 mRNA
ggccagggagcctcg

SEQ ID NO: 566 - DNA, 15 bp, Artificial Sequence
  h298-312 ASO for hRPS25 mRNA
tggccagggagcctc

SEQ ID NO: 567 - DNA, 15 bp, Artificial Sequence
  h299-313 ASO for hRPS25 mRNA
ctggccagggagcct

SEQ ID NO: 568 - DNA, 15 bp, Artificial Sequence
  h300-314 ASO for hRPS25 mRNA
cctggccagggagcc

SEQ ID NO: 569 - DNA, 15 bp, Artificial Sequence
  h321-335 ASO for hRPS25 mRNA
aaggagctcctgaag

SEQ ID NO: 570 - DNA, 15 bp, Artificial Sequence
  h322-336 ASO for hRPS25 mRNA
taaggagctcctgaa

SEQ ID NO: 571 - DNA, 15 bp, Artificial Sequence
  h323-337 ASO for hRPS25 mRNA
ctaaggagctcctga

SEQ ID NO: 572 - DNA, 15 bp, Artificial Sequence
  h324-338 ASO for hRPS25 mRNA
actaaggagctcctg

SEQ ID NO: 573 - DNA, 15 bp, Artificial Sequence
  h325-339 ASO for hRPS25 mRNA
tactaaggagctcct

SEQ ID NO: 574 - DNA, 15 bp, Artificial Sequence
  h326-340 ASO for hRPS25 mRNA
ttactaaggagctcc

SEQ ID NO: 575 - DNA, 15 bp, Artificial Sequence
  h327-341 ASO for hRPS25 mRNA
tttactaaggagctc

SEQ ID NO: 576 - DNA, 15 bp, Artificial Sequence
  h328-342 ASO for hRPS25 mRNA
ctttactaaggagct

SEQ ID NO: 577 - DNA, 15 bp, Artificial Sequence
  h329-343 ASO for hRPS25 mRNA
cctttactaaggagc

SEQ ID NO: 578 - DNA, 15 bp, Artificial Sequence
  h330-344 ASO for hRPS25 mRNA
tcctttactaaggag

SEQ ID NO: 579 - DNA, 15 bp, Artificial Sequence
  h331-345 ASO for hRPS25 mRNA
gtcctttactaagga

SEQ ID NO: 580 - DNA, 15 bp, Artificial Sequence
  h340-354 ASO for hRPS25 mRNA
gtttgataagtcctt

SEQ ID NO: 581 - DNA, 15 bp, Artificial Sequence
  h341-355 ASO for hRPS25 mRNA
agtttgataagtcct

SEQ ID NO: 582 - DNA, 15 bp, Artificial Sequence
  h342-356 ASO for hRPS25 mRNA
cagtttgataagtcc

SEQ ID NO: 583 - DNA, 15 bp, Artificial Sequence
  h343-357 ASO for hRPS25 mRNA
ccagtttgataagtc

SEQ ID NO: 584 - DNA, 15 bp, Artificial Sequence
  h344-358 ASO for hRPS25 mRNA
accagtttgataagt

SEQ ID NO: 585 - DNA, 15 bp, Artificial Sequence
  h365-379 ASO for hRPS25 mRNA
acttgagctctgtgc

SEQ ID NO: 586 - DNA, 15 bp, Artificial Sequence
  h375-389 ASO for hRPS25 mRNA
ggtgtaaattacttg

SEQ ID NO: 587 - DNA, 15 bp, Artificial Sequence
  h390-404 ASO for hRPS25 mRNA
acccttggtatttct

SEQ ID NO: 588 - DNA, 15 bp, Artificial Sequence
  h393-407 ASO for hRPS25 mRNA
tccacccttggtatt

SEQ ID NO: 589 - DNA, 15 bp, Artificial Sequence
  h394-408 ASO for hRPS25 mRNA
ctccacccttggtat

SEQ ID NO: 590 - DNA, 15 bp, Artificial Sequence
  h426-440 ASO for hRPS25 mRNA
tattcatgcatcttc

SEQ ID NO: 591 - DNA, 15 bp, Artificial Sequence
  h427-441 ASO for hRPS25 mRNA
ctattcatgcatctt

SEQ ID NO: 592 - DNA, 15 bp, Artificial Sequence
  h428-442 ASO for hRPS25 mRNA
cctattcatgcatct

SEQ ID NO: 593 - DNA, 15 bp, Artificial Sequence
  h429-443 ASO for hRPS25 mRNA
acctattcatgcatc

SEQ ID NO: 594 - DNA, 15 bp, Artificial Sequence
  h430-444 ASO for hRPS25 mRNA
gacctattcatgcat

SEQ ID NO: 595 - DNA, 15 bp, Artificial Sequence
  h431-445 ASO for hRPS25 mRNA
ggacctattcatgca

SEQ ID NO: 596 - DNA, 15 bp, Artificial Sequence
  h432-446 ASO for hRPS25 mRNA
tggacctattcatgc

SEQ ID NO: 597 - DNA, 15 bp, Artificial Sequence
  h433-447 ASO for hRPS25 mRNA
ttggacctattcatg

SEQ ID NO: 598 - DNA, 15 bp, Artificial Sequence
  h434-448 ASO for hRPS25 mRNA
gttggacctattcat

SEQ ID NO: 599 - DNA, 15 bp, Artificial Sequence
  h435-449 ASO for hRPS25 mRNA
ggttggacctattca

SEQ ID NO: 600 - DNA, 15 bp, Artificial Sequence
  h436-450 ASO for hRPS25 mRNA
tggttggacctattc

SEQ ID NO: 601 - DNA, 15 bp, Artificial Sequence
  h437-451 ASO for hRPS25 mRNA
ctggttggacctatt

SEQ ID NO: 602 - DNA, 15 bp, Artificial Sequence
  h438-452 ASO for hRPS25 mRNA
gctggttggacctat

SEQ ID NO: 603 - DNA, 15 bp, Artificial Sequence
  h439-453 ASO for hRPS25 mRNA
agctggttggaccta

SEQ ID NO: 604 - DNA, 15 bp, Artificial Sequence
  h440-454 ASO for hRPS25 mRNA
cagctggttggacct

SEQ ID NO: 605 - DNA, 15 bp, Artificial Sequence
  h441-455 ASO for hRPS25 mRNA
acagctggttggacc

SEQ ID NO: 606 - DNA, 15 bp, Artificial Sequence
  h442-456 ASO for hRPS25 mRNA
tacagctggttggac

SEQ ID NO: 607 - DNA, 15 bp, Artificial Sequence
  h443-457 ASO for hRPS25 mRNA
gtacagctggttgga

SEQ ID NO: 608 - DNA, 15 bp, Artificial Sequence
  h444-458 ASO for hRPS25 mRNA
tgtacagctggttgg

SEQ ID NO: 609 - DNA, 15 bp, Artificial Sequence
  h445-459 ASO for hRPS25 mRNA
atgtacagctggttg

SEQ ID NO: 610 - DNA, 15 bp, Artificial Sequence
  h446-460 ASO for hRPS25 mRNA
aatgtacagctggtt

SEQ ID NO: 611 - DNA, 15 bp, Artificial Sequence
  h447-461 ASO for hRPS25 mRNA
aaatgtacagctggt

SEQ ID NO: 612 - DNA, 15 bp, Artificial Sequence
  h448-462 ASO for hRPS25 mRNA
caaatgtacagctgg

SEQ ID NO: 613 - DNA, 15 bp, Artificial Sequence
  h449-463 ASO for hRPS25 mRNA
ccaaatgtacagctg

SEQ ID NO: 614 - DNA, 15 bp, Artificial Sequence
  h450-464 ASO for hRPS25 mRNA
tccaaatgtacagct

SEQ ID NO: 615 - DNA, 15 bp, Artificial Sequence
  h451-465 ASO for hRPS25 mRNA
ttccaaatgtacagc

SEQ ID NO: 616 - DNA, 15 bp, Artificial Sequence
  h452-466 ASO for hRPS25 mRNA
tttccaaatgtacag

SEQ ID NO: 617 - DNA, 15 bp, Artificial Sequence
  h453-467 ASO for hRPS25 mRNA
ttttccaaatgtaca

SEQ ID NO: 618 - DNA, 15 bp, Artificial Sequence
  h454-468 ASO for hRPS25 mRNA
tttttccaaatgtac

SEQ ID NO: 619 - DNA, 15 bp, Artificial Sequence
  h455-469 ASO for hRPS25 mRNA
atttttccaaatgta

SEQ ID NO: 620 - DNA, 19 bp, Artificial Sequence
  h123-141 ASO for hRPS25 mRNA
ccccggatttgttcactgg

SEQ ID NO: 621 - DNA, 17 bp, Artificial Sequence
  h124-140 ASO for hRPS25 mRNA
cccggatttgttcactg

SEQ ID NO: 622 - DNA, 16 bp, Artificial Sequence
  h125-140 ASO for hRPS25 mRNA
cccggatttgttcact

SEQ ID NO: 623 - DNA, 19 bp, Artificial Sequence
  h185-203 ASO for hRPS25 mRNA
gactaagttattgagcttg

SEQ ID NO: 624 - DNA, 16 bp, Artificial Sequence
  h186-201 ASO for hRPS25 mRNA
ctaagttattgagctt

SEQ ID NO: 625 - DNA, 17 bp, Artificial Sequence
  h186-202 ASO for hRPS25 mRNA
actaagttattgagctt

SEQ ID NO: 626 - DNA, 18 bp, Artificial Sequence
  h186-203 ASO for hRPS25 mRNA
gactaagttattgagctt

SEQ ID NO: 627 - DNA, 19 bp, Artificial Sequence
  h211-229 ASO for hRPS25 mRNA
ttatcataggtagctttgt

SEQ ID NO: 628 - DNA, 17 bp, Artificial Sequence
  h212-228 ASO for hRPS25 mRNA
tatcataggtagctttg

SEQ ID NO: 629 - DNA, 16 bp, Artificial Sequence
  h213-228 ASO for hRPS25 mRNA
tatcataggtagcttt

SEQ ID NO: 630 - DNA, 16 bp, Artificial Sequence
  h214-229 ASO for hRPS25 mRNA
ttatcataggtagctt

SEQ ID NO: 631 - DNA, 16 bp, Artificial Sequence
  h259-274 ASO for hRPS25 mRNA
acagctggggttataa

SEQ ID NO: 632 - DNA, 17 bp, Artificial Sequence
  h263-279 ASO for hRPS25 mRNA
agaccacagctggggtt

SEQ ID NO: 633 - DNA, 17 bp, Artificial Sequence
  h264-280 ASO for hRPS25 mRNA
gagaccacagctggggt

SEQ ID NO: 634 - DNA, 15 bp, Artificial Sequence
  h265-279 ASO for hRPS25 mRNA
agaccacagctgggg

SEQ ID NO: 635 - DNA, 15 bp, Artificial Sequence
  h266-280 ASO for hRPS25 mRNA
gagaccacagctggg

SEQ ID NO: 636 - DNA, 15 bp, Artificial Sequence
  h267-281 ASO for hRPS25 mRNA
agagaccacagctgg

SEQ ID NO: 637 - DNA, 15 bp, Artificial Sequence
  h268-282 ASO for hRPS25 mRNA
cagagaccacagctg

SEQ ID NO: 638 - DNA, 17 bp, Artificial Sequence
  h295-311 ASO for hRPS25 mRNA
ggccagggagcctcgaa

SEQ ID NO: 639 - DNA, 16 bp, Artificial Sequence
  h296-311 ASO for hRPS25 mRNA
ggccagggagcctcga

SEQ ID NO: 640 - DNA, 17 bp, Artificial Sequence
  h300-316 ASO for hRPS25 mRNA
gccctggccagggagcc

SEQ ID NO: 641 - DNA, 15 bp, Artificial Sequence
  h301-315 ASO for hRPS25 mRNA
ccctggccagggagc

SEQ ID NO: 642 - DNA, 15 bp, Artificial Sequence
  h302-316 ASO for hRPS25 mRNA
gccctggccagggag

SEQ ID NO: 643 - DNA, 15 bp, Artificial Sequence
  h303-317 ASO for hRPS25 mRNA
tgccctggccaggga

SEQ ID NO: 644 - DNA, 15 bp, Artificial Sequence
  h304-318 ASO for hRPS25 mRNA
ctgccctggccaggg

SEQ ID NO: 645 - DNA, 17 bp, Artificial Sequence
  h322-338 ASO for hRPS25 mRNA
actaaggagctcctgaa

SEQ ID NO: 646 - DNA, 19 bp, Artificial Sequence
  h324-342 ASO for hRPS25 mRNA
ctttactaaggagctcctg

SEQ ID NO: 647 - DNA, 16 bp, Artificial Sequence
  h325-340 ASO for hRPS25 mRNA
ttactaaggagctcct

SEQ ID NO: 648 - DNA, 17 bp, Artificial Sequence
  h325-341 ASO for hRPS25 mRNA
tttactaaggagctcct

SEQ ID NO: 649 - DNA, 16 bp, Artificial Sequence
  h326-341 ASO for hRPS25 mRNA
tttactaaggagctcc

SEQ ID NO: 650 - DNA, 17 bp, Artificial Sequence
  h429-445 ASO for hRPS25 mRNA
ggacctattcatgcatc

SEQ ID NO: 651 - DNA, 17 bp, Artificial Sequence
  h430-446 ASO for hRPS25 mRNA
tggacctattcatgcat

SEQ ID NO: 652 - DNA, 17 bp, Artificial Sequence
  h434-450 ASO for hRPS25 mRNA
tggttggacctattcat

SEQ ID NO: 653 - DNA, 16 bp, Artificial Sequence
  h439-454 ASO for hRPS25 mRNA
cagctggttggaccta

SEQ ID NO: 654 - DNA, 17 bp, Artificial Sequence
  h439-455 ASO for hRPS25 mRNA
acagctggttggaccta

SEQ ID NO: 655 - DNA, 17 bp, Artificial Sequence
  h441-457 ASO for hRPS25 mRNA
gtacagctggttggacc

SEQ ID NO: 656 - DNA, 16 bp, Artificial Sequence
  h442-457 ASO for hRPS25 mRNA
gtacagctggttggac

SEQ ID NO: 657 - DNA, 17 bp, Artificial Sequence
  h442-458 ASO for hRPS25 mRNA
tgtacagctggttggac

SEQ ID NO: 658 - DNA, 18 bp, Artificial Sequence
  h442-459 ASO for hRPS25 mRNA
atgtacagctggttggac

SEQ ID NO: 659 - DNA, 19 bp, Artificial Sequence
  h442-460 ASO for hRPS25 mRNA
aatgtacagctggttggac

SEQ ID NO: 660 - DNA, 16 bp, Artificial Sequence
  h443-458 ASO for hRPS25 mRNA
tgtacagctggttgga

SEQ ID NO: 661 - DNA, 17 bp, Artificial Sequence
  h443-459 ASO for hRPS25 mRNA
atgtacagctggttgga

SEQ ID NO: 662 - DNA, 18 bp, Artificial Sequence
  h443-460 ASO for hRPS25 mRNA
aatgtacagctggttgga

SEQ ID NO: 663 - DNA, 19 bp, Artificial Sequence
  h447-465 ASO for hRPS25 mRNA
ttccaaatgtacagctggt

SEQ ID NO: 664 - DNA, 18 bp, Artificial Sequence
  h448-465 ASO for hRPS25 mRNA
ttccaaatgtacagctgg

SEQ ID NO: 665 - DNA, 19 bp, Artificial Sequence
  h448-466 ASO for hRPS25 mRNA
tttccaaatgtacagctgg

SEQ ID NO: 666 - DNA, 17 bp, Artificial Sequence
  h449-465 ASO for hRPS25 mRNA
ttccaaatgtacagctg

SEQ ID NO: 667 - DNA, 18 bp, Artificial Sequence
  h449-466 ASO for hRPS25 mRNA
tttccaaatgtacagctg

SEQ ID NO: 668 - DNA, 19 bp, Artificial Sequence
  h449-467 ASO for hRPS25 mRNA
ttttccaaatgtacagctg

SEQ ID NO: 669 - DNA, 16 bp, Artificial Sequence
  h450-465 ASO for hRPS25 mRNA
ttccaaatgtacagct

SEQ ID NO: 670 - DNA, 17 bp, Artificial Sequence
  h450-466 ASO for hRPS25 mRNA
tttccaaatgtacagct

SEQ ID NO: 671 - DNA, 18 bp, Artificial Sequence
  h450-467 ASO for hRPS25 mRNA
ttttccaaatgtacagct

SEQ ID NO: 672 - DNA, 19 bp, Artificial Sequence
  h450-468 ASO for hRPS25 mRNA
tttttccaaatgtacagct

SEQ ID NO: 673 - DNA, 16 bp, Artificial Sequence
  h451-466 ASO for hRPS25 mRNA
tttccaaatgtacagc

SEQ ID NO: 674 - DNA, 17 bp, Artificial Sequence
  h451-467 ASO for hRPS25 mRNA
ttttccaaatgtacagc

SEQ ID NO: 675 - DNA, 18 bp, Artificial Sequence
  h451-468 ASO for hRPS25 mRNA
tttttccaaatgtacagc

SEQ ID NO: 676 - DNA, 19 bp, Artificial Sequence
  h451-469 ASO for hRPS25 mRNA
atttttccaaatgtacagc

SEQ ID NO: 677 - DNA, 15 bp, Artificial Sequence
  hp1-15 ASO for hRPS25 pre-mRNA
cggacaaaaaggaag

SEQ ID NO: 678 - DNA, 15 bp, Artificial Sequence
  hp72-86 ASO for hRPS25 pre-mRNA
ttcacacccctgaag

SEQ ID NO: 679 - DNA, 15 bp, Artificial Sequence
  hp73-87 ASO for hRPS25 pre-mRNA
cttcacacccctgaa

SEQ ID NO: 680 - DNA, 15 bp, Artificial Sequence
  hp74-88 ASO for hRPS25 pre-mRNA
acttcacacccctga

SEQ ID NO: 681 - DNA, 15 bp, Artificial Sequence
  hp75-89 ASO for hRPS25 pre-mRNA
gacttcacacccctg

SEQ ID NO: 682 - DNA, 15 bp, Artificial Sequence
  hp76-90 ASO for hRPS25 pre-mRNA
cgacttcacacccct

SEQ ID NO: 683 - DNA, 15 bp, Artificial Sequence
  hp231-245 ASO for hRPS25 pre-mRNA
tcccctaatactgcg

SEQ ID NO: 684 - DNA, 15 bp, Artificial Sequence
  hp232-246 ASO for hRPS25 pre-mRNA
gtcccctaatactgc

SEQ ID NO: 685 - DNA, 15 bp, Artificial Sequence
  hp233-247 ASO for hRPS25 pre-mRNA
agtcccctaatactg

SEQ ID NO: 686 - DNA, 15 bp, Artificial Sequence
  hp261-275 ASO for hRPS25 pre-mRNA
atgcaaccaggtcct

SEQ ID NO: 687 - DNA, 15 bp, Artificial Sequence
  hp262-276 ASO for hRPS25 pre-mRNA
aatgcaaccaggtcc

SEQ ID NO: 688 - DNA, 15 bp, Artificial Sequence
  hp278-292 ASO for hRPS25 pre-mRNA
gtaggagggcagcgg

SEQ ID NO: 689 - DNA, 15 bp, Artificial Sequence
  hp279-293 ASO for hRPS25 pre-mRNA
tgtaggagggcagcg

SEQ ID NO: 690 - DNA, 15 bp, Artificial Sequence
  hp280-294 ASO for hRPS25 pre-mRNA
ctgtaggagggcagc

SEQ ID NO: 691 - DNA, 15 bp, Artificial Sequence
  hp390-404 ASO for hRPS25 pre-mRNA
ggtcttatttctacc

SEQ ID NO: 692 - DNA, 15 bp, Artificial Sequence
  hp392-406 ASO for hRPS25 pre-mRNA
gaggtcttatttcta

SEQ ID NO: 693 - DNA, 15 bp, Artificial Sequence
  hp417-431 ASO for hRPS25 pre-mRNA
agagttacccctagt

SEQ ID NO: 694 - DNA, 15 bp, Artificial Sequence
  hp418-432 ASO for hRPS25 pre-mRNA
gagagttacccctag

SEQ ID NO: 695 - DNA, 15 bp, Artificial Sequence
  hp419-433 ASO for hRPS25 pre-mRNA
agagagttaccccta

SEQ ID NO: 696 - DNA, 15 bp, Artificial Sequence
  hp420-434 ASO for hRPS25 pre-mRNA
gagagagttacccct

SEQ ID NO: 697 - DNA, 15 bp, Artificial Sequence
  hp421-435 ASO for hRPS25 pre-mRNA
cgagagagttacccc

SEQ ID NO: 698 - DNA, 15 bp, Artificial Sequence
  hp422-436 ASO for hRPS25 pre-mRNA
acgagagagttaccc

SEQ ID NO: 699 - DNA, 15 bp, Artificial Sequence
  hp423-437 ASO for hRPS25 pre-mRNA
tacgagagagttacc

SEQ ID NO: 700 - DNA, 15 bp, Artificial Sequence
  hp445-459 ASO for hRPS25 pre-mRNA
aagttacctattact

SEQ ID NO: 701 - DNA, 15 bp, Artificial Sequence
  hp446-460 ASO for hRPS25 pre-mRNA
caagttacctattac

SEQ ID NO: 702 - DNA, 15 bp, Artificial Sequence
  hp447-461 ASO for hRPS25 pre-mRNA
acaagttacctatta

SEQ ID NO: 703 - DNA, 15 bp, Artificial Sequence
  hp448-462 ASO for hRPS25 pre-mRNA
tacaagttacctatt

SEQ ID NO: 704 - DNA, 15 bp, Artificial Sequence
  hp458-472 ASO for hRPS25 pre-mRNA
ccacttactatacaa

SEQ ID NO: 705 - DNA, 15 bp, Artificial Sequence
  hp460-474 ASO for hRPS25 pre-mRNA
aaccacttactatac

SEQ ID NO: 706 - DNA, 15 bp, Artificial Sequence
  hp461-475 ASO for hRPS25 pre-mRNA
aaaccacttactata

SEQ ID NO: 707 - DNA, 15 bp, Artificial Sequence
  hp510-524 ASO for hRPS25 pre-mRNA
gacgggaagataaac

SEQ ID NO: 708 - DNA, 15 bp, Artificial Sequence
  hp561-575 ASO for hRPS25 pre-mRNA
tcgcacaacagaccc

SEQ ID NO: 709 - DNA, 15 bp, Artificial Sequence
  hp562-576 ASO for hRPS25 pre-mRNA
ttcgcacaacagacc

SEQ ID NO: 710 - DNA, 15 bp, Artificial Sequence
  hp589-603 ASO for hRPS25 pre-mRNA
taacacagcaggcac

SEQ ID NO: 711 - DNA, 15 bp, Artificial Sequence
  hp605-619 ASO for hRPS25 pre-mRNA
ctagatcagttaaaa

SEQ ID NO: 712 - DNA, 15 bp, Artificial Sequence
  hp606-620 ASO for hRPS25 pre-mRNA
actagatcagttaaa

SEQ ID NO: 713 - DNA, 15 bp, Artificial Sequence
  hp626-640 ASO for hRPS25 pre-mRNA
tcaaacaggggccga

SEQ ID NO: 714 - DNA, 15 bp, Artificial Sequence
  hp627-641 ASO for hRPS25 pre-mRNA
ttcaaacaggggccg

SEQ ID NO: 715 - DNA, 15 bp, Artificial Sequence
  hp628-642 ASO for hRPS25 pre-mRNA
cttcaaacaggggcc

SEQ ID NO: 716 - DNA, 15 bp, Artificial Sequence
  hp629-643 ASO for hRPS25 pre-mRNA
ccttcaaacaggggc

SEQ ID NO: 717 - DNA, 15 bp, Artificial Sequence
  hp632-646 ASO for hRPS25 pre-mRNA
tggccttcaaacagg

SEQ ID NO: 718 - DNA, 15 bp, Artificial Sequence
  hp633-647 ASO for hRPS25 pre-mRNA
ttggccttcaaacag

SEQ ID NO: 719 - DNA, 15 bp, Artificial Sequence
  hp634-648 ASO for hRPS25 pre-mRNA
tttggccttcaaaca

SEQ ID NO: 720 - DNA, 15 bp, Artificial Sequence
  hp654-668 ASO for hRPS25 pre-mRNA
aaaaaaaacaccgac

SEQ ID NO: 721 - DNA, 15 bp, Artificial Sequence
  hp681-695 ASO for hRPS25 pre-mRNA
aattacacattacta

SEQ ID NO: 722 - DNA, 15 bp, Artificial Sequence
  hp696-710 ASO for hRPS25 pre-mRNA
ccgttatcaaggata

SEQ ID NO: 723 - DNA, 15 bp, Artificial Sequence
  hp697-711 ASO for hRPS25 pre-mRNA
accgttatcaaggat

SEQ ID NO: 724 - DNA, 15 bp, Artificial Sequence
  hp761-775 ASO for hRPS25 pre-mRNA
gttagtatttctggc

SEQ ID NO: 725 - DNA, 15 bp, Artificial Sequence
  hp762-776 ASO for hRPS25 pre-mRNA
agttagtatttctgg

SEQ ID NO: 726 - DNA, 15 bp, Artificial Sequence
  hp764-778 ASO for hRPS25 pre-mRNA
caagttagtatttct

SEQ ID NO: 727 - DNA, 15 bp, Artificial Sequence
  hp1034-1048 ASO for hRPS25 pre-mRNA
atgcttaacatggtc

SEQ ID NO: 728 - DNA, 15 bp, Artificial Sequence
  hp1035-1049 ASO for hRPS25 pre-mRNA
gatgcttaacatggt

SEQ ID NO: 729 - DNA, 15 bp, Artificial Sequence
  hp1103-1117 ASO for hRPS25 pre-mRNA
ttactaacagccaat

SEQ ID NO: 730 - DNA, 15 bp, Artificial Sequence
  hp1104-1118 ASO for hRPS25 pre-mRNA
attactaacagccaa

SEQ ID NO: 731 - DNA, 15 bp, Artificial Sequence
  hp1105-1119 ASO for hRPS25 pre-mRNA
cattactaacagcca

SEQ ID NO: 732 - DNA, 15 bp, Artificial Sequence
  hp1106-1120 ASO for hRPS25 pre-mRNA
acattactaacagcc

SEQ ID NO: 733 - DNA, 15 bp, Artificial Sequence
  hp1107-1121 ASO for hRPS25 pre-mRNA
tacattactaacagc

SEQ ID NO: 734 - DNA, 15 bp, Artificial Sequence
  hp1108-1122 ASO for hRPS25 pre-mRNA
ttacattactaacag

SEQ ID NO: 735 - DNA, 15 bp, Artificial Sequence
  hp1110-1124 ASO for hRPS25 pre-mRNA
aattacattactaac

SEQ ID NO: 736 - DNA, 15 bp, Artificial Sequence
  hp1128-1142 ASO for hRPS25 pre-mRNA
tcaggagtaagacgt

SEQ ID NO: 737 - DNA, 15 bp, Artificial Sequence
  hp1129-1143 ASO for hRPS25 pre-mRNA
atcaggagtaagacg

SEQ ID NO: 738 - DNA, 15 bp, Artificial Sequence
  hp1196-1210 ASO for hRPS25 pre-mRNA
gcttcactaaactgc

SEQ ID NO: 739 - DNA, 15 bp, Artificial Sequence
  hp1197-1211 ASO for hRPS25 pre-mRNA
ggcttcactaaactg

SEQ ID NO: 740 - DNA, 15 bp, Artificial Sequence
  hp1217-1231 ASO for hRPS25 pre-mRNA
cgaaacataaaagat

SEQ ID NO: 741 - DNA, 15 bp, Artificial Sequence
  hp1218-1232 ASO for hRPS25 pre-mRNA
tcgaaacataaaaga

SEQ ID NO: 742 - DNA, 15 bp, Artificial Sequence
  hp1219-1233 ASO for hRPS25 pre-mRNA
ctcgaaacataaaag

SEQ ID NO: 743 - DNA, 15 bp, Artificial Sequence
  hp1398-1412 ASO for hRPS25 pre-mRNA
gtggaattatggtaa

SEQ ID NO: 744 - DNA, 15 bp, Artificial Sequence
  hp1399-1413 ASO for hRPS25 pre-mRNA
tgtggaattatggta

SEQ ID NO: 745 - DNA, 15 bp, Artificial Sequence
  hp1402-1416 ASO for hRPS25 pre-mRNA
tattgtggaattatg

SEQ ID NO: 746 - DNA, 15 bp, Artificial Sequence
  hp1408-1422 ASO for hRPS25 pre-mRNA
ccttattattgtgga

SEQ ID NO: 747 - DNA, 15 bp, Artificial Sequence
  hp1409-1423 ASO for hRPS25 pre-mRNA
gccttattattgtgg

SEQ ID NO: 748 - DNA, 15 bp, Artificial Sequence
  hp1410-1424 ASO for hRPS25 pre-mRNA
agccttattattgtg

SEQ ID NO: 749 - DNA, 15 bp, Artificial Sequence
  hp1411-1425 ASO for hRPS25 pre-mRNA
gagccttattattgt

SEQ ID NO: 750 - DNA, 15 bp, Artificial Sequence
  hp1412-1426 ASO for hRPS25 pre-mRNA
tgagccttattattg

SEQ ID NO: 751 - DNA, 15 bp, Artificial Sequence
  hp1478-1492 ASO for hRPS25 pre-mRNA
cgttgattcacccgc

SEQ ID NO: 752 - DNA, 15 bp, Artificial Sequence
  hp1480-1494 ASO for hRPS25 pre-mRNA
tccgttgattcaccc

SEQ ID NO: 753 - DNA, 15 bp, Artificial Sequence
  hp1715-1729 ASO for hRPS25 pre-mRNA
gctccattatcttcc

SEQ ID NO: 754 - DNA, 15 bp, Artificial Sequence
  hp1749-1763 ASO for hRPS25 pre-mRNA
cgatcatctatcctt

SEQ ID NO: 755 - DNA, 15 bp, Artificial Sequence
  hp1750-1764 ASO for hRPS25 pre-mRNA
acgatcatctatcct

SEQ ID NO: 756 - DNA, 15 bp, Artificial Sequence
  hp1751-1765 ASO for hRPS25 pre-mRNA
aacgatcatctatcc

SEQ ID NO: 757 - DNA, 15 bp, Artificial Sequence
  hp1763-1777 ASO for hRPS25 pre-mRNA
atcctagtttttaac

SEQ ID NO: 758 - DNA, 15 bp, Artificial Sequence
  hp1793-1807 ASO for hRPS25 pre-mRNA
attgcttaatctgac

SEQ ID NO: 759 - DNA, 15 bp, Artificial Sequence
  hp1885-1899 ASO for hRPS25 pre-mRNA
atggtcttaaaactc

SEQ ID NO: 760 - DNA, 15 bp, Artificial Sequence
  hp1887-1901 ASO for hRPS25 pre-mRNA
gaatggtcttaaaac

SEQ ID NO: 761 - DNA, 15 bp, Artificial Sequence
  hp2047-2061 ASO for hRPS25 pre-mRNA
gtttgttttggccgg

SEQ ID NO: 762 - DNA, 15 bp, Artificial Sequence
  hp2048-2062 ASO for hRPS25 pre-mRNA
ggtttgttttggccg

SEQ ID NO: 763 - DNA, 15 bp, Artificial Sequence
  hp2049-2063 ASO for hRPS25 pre-mRNA
aggtttgttttggcc

SEQ ID NO: 764 - DNA, 15 bp, Artificial Sequence
  hp2121-2135 ASO for hRPS25 pre-mRNA
gaattggtggttgca

SEQ ID NO: 765 - DNA, 15 bp, Artificial Sequence
  hp2122-2136 ASO for hRPS25 pre-mRNA
ggaattggtggttgc

SEQ ID NO: 766 - DNA, 15 bp, Artificial Sequence
  hp2123-2137 ASO for hRPS25 pre-mRNA
aggaattggtggttg

SEQ ID NO: 767 - DNA, 15 bp, Artificial Sequence
  hp2124-2138 ASO for hRPS25 pre-mRNA
caggaattggtggtt

SEQ ID NO: 768 - DNA, 15 bp, Artificial Sequence
  hp2260-2274 ASO for hRPS25 pre-mRNA
ggtaaggagttgcac

SEQ ID NO: 769 - DNA, 15 bp, Artificial Sequence
  hp2261-2275 ASO for hRPS25 pre-mRNA
aggtaaggagttgca

SEQ ID NO: 770 - DNA, 15 bp, Artificial Sequence
  hp2262-2276 ASO for hRPS25 pre-mRNA
gaggtaaggagttgc

SEQ ID NO: 771 - DNA, 15 bp, Artificial Sequence
  hp2268-2282 ASO for hRPS25 pre-mRNA
tagcttgaggtaagg

SEQ ID NO: 772 - DNA, 15 bp, Artificial Sequence
  hp2269-2283 ASO for hRPS25 pre-mRNA
atagcttgaggtaag

SEQ ID NO: 773 - DNA, 15 bp, Artificial Sequence
  hp2271-2285 ASO for hRPS25 pre-mRNA
agatagcttgaggta

SEQ ID NO: 774 - DNA, 15 bp, Artificial Sequence
  hp2277-2291 ASO for hRPS25 pre-mRNA
acgggcagatagctt

SEQ ID NO: 775 - DNA, 15 bp, Artificial Sequence
  hp2339-2353 ASO for hRPS25 pre-mRNA
gtaaggtttttggct

SEQ ID NO: 776 - DNA, 15 bp, Artificial Sequence
  hp2341-2355 ASO for hRPS25 pre-mRNA
tagtaaggtttttgg

SEQ ID NO: 777 - DNA, 15 bp, Artificial Sequence
  hp2342-2356 ASO for hRPS25 pre-mRNA
ctagtaaggtttttg

SEQ ID NO: 778 - DNA, 15 bp, Artificial Sequence
  hp2386-2400 ASO for hRPS25 pre-mRNA
agagaatagcacgat

SEQ ID NO: 779 - DNA, 15 bp, Artificial Sequence
  hp2406-2420 ASO for hRPS25 pre-mRNA
gtttgataagtccta

SEQ ID NO: 780 - DNA, 15 bp, Artificial Sequence
  hp2538-2552 ASO for hRPS25 pre-mRNA
tttgtatctacctcc

SEQ ID NO: 781 - DNA, 15 bp, Artificial Sequence
  hp2540-2554 ASO for hRPS25 pre-mRNA
gctttgtatctacct

SEQ ID NO: 782 - DNA, 15 bp, Artificial Sequence
  hp2541-2555 ASO for hRPS25 pre-mRNA
agctttgtatctacc

SEQ ID NO: 783 - DNA, 15 bp, Artificial Sequence
  hp2585-2599 ASO for hRPS25 pre-mRNA
ctggttggacctgta

SEQ ID NO: 784 - DNA, 15 bp, Artificial Sequence
  hp2586-2600 ASO for hRPS25 pre-mRNA
gctggttggacctgt

SEQ ID NO: 785 - DNA, 15 bp, Artificial Sequence
  hp2587-2601 ASO for hRPS25 pre-mRNA
agctggttggacctg

SEQ ID NO: 786 - DNA, 15 bp, Artificial Sequence
  hp2583-2597 ASO for hRPS25 pre-mRNA
ggttggacctgtaaa

SEQ ID NO: 787 - DNA, 15 bp, Artificial Sequence
  hp2584-2598 ASO for hRPS25 pre-mRNA
tggttggacctgtaa

SEQ ID NO: 788 - DNA, 703 bp, Artificial Sequence
  Myc, Flag, V5
gctagccaccatggcgaccctggaaaagatgatgaaggccttcgagtccctcaagtccttccagcagcagcagcagcagcagcagcagcagcagcagcagcagcagcagcagcagcagcagcagcagcagcagcagcagcagcagcagcagcagcagcagcagcagcagcagcagcagcagcagcagcagcagcagcagcagcagcagcagcagcagcagcagcagcagcagcagcagcagcagcagcagcagcagcagcagcagcagcagcagcagcagcagcagcagcagcagcagcagcagcagcagcagcagcagcagcagcagcagcagcagcagcagcagcagcagcagcagcagcagcagcagcagcagcagcagcagcagcagcagcagcagcagcagcagcagcagcagcagccgccaccgccgccgccgccgccgccgcctcctcagcttcctcagccgccgccgcaggcacagccgctgctgcctcagccgcagccgcccccgccgccgcccccgccgccacccggcccggctgtggctgtggagccgcaagaattcggaggagatatcgaacaaaaactcatctcagaagaggatctgtgactacaaagacgacgacgacaagcggtaagcctatccctaaccctctcctcggtctcgattctacgtagctcgagtctagagggcccgttt